European Patent Specification EP 2 855 667 B1, published August 9, 2023. Title: Methods for engineering allogeneic and immunosuppressive resistant T cell for immunotherapy. Applicant: GALETTO ROMAN GROSSE STEPHANIE GOUBLE AGNES MANNIOUI CECILE POIROT LAURENT SMITH JULIANNE SCHARENBERG ANDREW. The sequence listing filed with the application follows.

SEQUENCE LISTING (126 sequences)

SEQ ID NO: 1 - DNA, 49 bp, Artificialsequence
  GRex2
tattcactgatggactccaaagaatcattaactcctggtagagaagaaa

SEQ ID NO: 2 - DNA, 49 bp, Artificialsequence
  GRex3T2
tgcctggtgtgctctgatgaagcttcaggatgtcattatggagtcttaa

SEQ ID NO: 3 - DNA, 49 bp, Artificialsequence
  GRex3T4
tgctctgatgaagcttcaggatgtcattatggagtcttaacttgtggaa

SEQ ID NO: 4 - DNA, 49 bp, Artificialsequence
  GRex5T1
tggtgtcactgttggaggttattgaacctgaagtgttatatgcaggata

SEQ ID NO: 5 - DNA, 49 bp, Artificialsequence
  GRex5T2
tatgatagctctgttccagactcaacttggaggatcatgactacgctca

SEQ ID NO: 6 - DNA, 49 bp, Artificialsequence
  GRex5T3
ttatatgcaggatatgatagctctgttccagactcaacttggaggatca

SEQ ID NO: 7 - protein, 530 aa, Artificialsequence
  Repeat-GRex2-LPT9-L1
LTPEQVVAIASNIGGKQALETVQALLPVLCQAHGLTPQQVVAIASNGGGKQALETVQRLLPVLCQAHGLTPQQVVAIASNGGGKQALETVQRLLPVLCQAHGLTPEQVVAIASHDGGKQALETVQRLLPVLCQAHGLTPEQVVAIASNIGGKQALETVQALLPVLCQAHGLTPEQVVAIASHDGGKQALETVQRLLPVLCQAHGLTPQQVVAIASNGGGKQALETVQRLLPVLCQAHGLTPQQVVAIASNNGGKQALETVQRLLPVLCQAHGLTPEQVVAIASNIGGKQALETVQALLPVLCQAHGLTPQQVVAIASNGGGKQALETVQRLLPVLCQAHGLTPQQVVAIASNNGGKQALETVQRLLPVLCQAHGLTPQQVVAIASNNGGKQALETVQRLLPVLCQAHGLTPEQVVAIASNIGGKQALETVQALLPVLCQAHGLTPEQVVAIASHDGGKQALETVQRLLPVLCQAHGLTPQQVVAIASNGGGKQALETVQRLLPVLCQAHGLTPQQVVAIASNGGGRPALE

SEQ ID NO: 8 - protein, 530 aa, Artificialsequence
  Repeat-GRex2-LPT9-R1
LTPQQVVAIASNGGGKQALETVQRLLPVLCQAHGLTPQQVVAIASNGGGKQALETVQRLLPVLCQAHGLTPEQVVAIASHDGGKQALETVQRLLPVLCQAHGLTPQQVVAIASNGGGKQALETVQRLLPVLCQAHGLTPQQVVAIASNGGGKQALETVQRLLPVLCQAHGLTPEQVVAIASHDGGKQALETVQRLLPVLCQAHGLTPQQVVAIASNGGGKQALETVQRLLPVLCQAHGLTPEQVVAIASHDGGKQALETVQRLLPVLCQAHGLTPQQVVAIASNGGGKQALETVQRLLPVLCQAHGLTPEQVVAIASNIGGKQALETVQALLPVLCQAHGLTPEQVVAIASHDGGKQALETVQRLLPVLCQAHGLTPEQVVAIASHDGGKQALETVQRLLPVLCQAHGLTPEQVVAIASNIGGKQALETVQALLPVLCQAHGLTPQQVVAIASNNGGKQALETVQRLLPVLCQAHGLTPQQVVAIASNNGGKQALETVQRLLPVLCQAHGLTPQQVVAIASNGGGRPALE

SEQ ID NO: 9 - protein, 530 aa, Artificialsequence
  Repeat-GRex3T2-L1
LTPQQVVAIASNNGGKQALETVQRLLPVLCQAHGLTPEQVVAIASHDGGKQALETVQRLLPVLCQAHGLTPEQVVAIASHDGGKQALETVQRLLPVLCQAHGLTPQQVVAIASNGGGKQALETVQRLLPVLCQAHGLTPQQVVAIASNNGGKQALETVQRLLPVLCQAHGLTPQQVVAIASNNGGKQALETVQRLLPVLCQAHGLTPQQVVAIASNGGGKQALETVQRLLPVLCQAHGLTPQQVVAIASNNGGKQALETVQRLLPVLCQAHGLTPQQVVAIASNGGGKQALETVQRLLPVLCQAHGLTPQQVVAIASNNGGKQALETVQRLLPVLCQAHGLTPEQVVAIASHDGGKQALETVQRLLPVLCQAHGLTPQQVVAIASNGGGKQALETVQRLLPVLCQAHGLTPEQVVAIASHDGGKQALETVQRLLPVLCQAHGLTPQQVVAIASNGGGKQALETVQRLLPVLCQAHGLTPQQVVAIASNNGGKQALETVQRLLPVLCQAHGLTPQQVVAIASNGGGRPALE

SEQ ID NO: 10 - protein, 530 aa, Artificialsequence
  Repeat-GRex3T2-R1
LTPQQVVAIASNGGGKQALETVQRLLPVLCQAHGLTPEQVVAIASNIGGKQALETVQALLPVLCQAHGLTPEQVVAIASNIGGKQALETVQALLPVLCQAHGLTPQQVVAIASNNGGKQALETVQRLLPVLCQAHGLTPEQVVAIASNIGGKQALETVQALLPVLCQAHGLTPEQVVAIASHDGGKQALETVQRLLPVLCQAHGLTPQQVVAIASNGGGKQALETVQRLLPVLCQAHGLTPEQVVAIASHDGGKQALETVQRLLPVLCQAHGLTPEQVVAIASHDGGKQALETVQRLLPVLCQAHGLTPEQVVAIASNIGGKQALETVQALLPVLCQAHGLTPQQVVAIASNGGGKQALETVQRLLPVLCQAHGLTPEQVVAIASNIGGKQALETVQALLPVLCQAHGLTPEQVVAIASNIGGKQALETVQALLPVLCQAHGLTPQQVVAIASNGGGKQALETVQRLLPVLCQAHGLTPQQVVAIASNNGGKQALETVQRLLPVLCQAHGLTPQQVVAIASNGGGRPALE

SEQ ID NO: 11 - protein, 530 aa, Artificialsequence
  Repeat-GRex3T4-L1
LTPQQVVAIASNNGGKQALETVQRLLPVLCQAHGLTPEQVVAIASHDGGKQALETVQRLLPVLCQAHGLTPQQVVAIASNGGGKQALETVQRLLPVLCQAHGLTPEQVVAIASHDGGKQALETVQRLLPVLCQAHGLTPQQVVAIASNGGGKQALETVQRLLPVLCQAHGLTPQQVVAIASNNGGKQALETVQRLLPVLCQAHGLTPEQVVAIASNIGGKQALETVQALLPVLCQAHGLTPQQVVAIASNGGGKQALETVQRLLPVLCQAHGLTPQQVVAIASNNGGKQALETVQRLLPVLCQAHGLTPEQVVAIASNIGGKQALETVQALLPVLCQAHGLTPEQVVAIASNIGGKQALETVQALLPVLCQAHGLTPQQVVAIASNNGGKQALETVQRLLPVLCQAHGLTPEQVVAIASHDGGKQALETVQRLLPVLCQAHGLTPQQVVAIASNGGGKQALETVQRLLPVLCQAHGLTPQQVVAIASNGGGKQALETVQRLLPVLCQAHGLTPQQVVAIASNGGGRPALE

SEQ ID NO: 12 - protein, 530 aa, Artificialsequence
  Repeat-GRex3T4-R1
LTPQQVVAIASNGGGKQALETVQRLLPVLCQAHGLTPEQVVAIASHDGGKQALETVQRLLPVLCQAHGLTPEQVVAIASHDGGKQALETVQRLLPVLCQAHGLTPEQVVAIASNIGGKQALETVQALLPVLCQAHGLTPEQVVAIASHDGGKQALETVQRLLPVLCQAHGLTPEQVVAIASNIGGKQALETVQALLPVLCQAHGLTPEQVVAIASNIGGKQALETVQALLPVLCQAHGLTPQQVVAIASNNGGKQALETVQRLLPVLCQAHGLTPQQVVAIASNGGGKQALETVQRLLPVLCQAHGLTPQQVVAIASNGGGKQALETVQRLLPVLCQAHGLTPEQVVAIASNIGGKQALETVQALLPVLCQAHGLTPEQVVAIASNIGGKQALETVQALLPVLCQAHGLTPQQVVAIASNNGGKQALETVQRLLPVLCQAHGLTPEQVVAIASNIGGKQALETVQALLPVLCQAHGLTPEQVVAIASHDGGKQALETVQRLLPVLCQAHGLTPQQVVAIASNGGGRPALE

SEQ ID NO: 13 - protein, 530 aa, Artificialsequence
  Repeat-GRex5T1-LPT8-L1
LTPQQVVAIASNNGGKQALETVQRLLPVLCQAHGLTPQQVVAIASNNGGKQALETVQRLLPVLCQAHGLTPQQVVAIASNGGGKQALETVQRLLPVLCQAHGLTPQQVVAIASNNGGKQALETVQRLLPVLCQAHGLTPQQVVAIASNGGGKQALETVQRLLPVLCQAHGLTPEQVVAIASHDGGKQALETVQRLLPVLCQAHGLTPEQVVAIASNIGGKQALETVQALLPVLCQAHGLTPEQVVAIASHDGGKQALETVQRLLPVLCQAHGLTPQQVVAIASNGGGKQALETVQRLLPVLCQAHGLTPQQVVAIASNNGGKQALETVQRLLPVLCQAHGLTPQQVVAIASNGGGKQALETVQRLLPVLCQAHGLTPQQVVAIASNGGGKQALETVQRLLPVLCQAHGLTPQQVVAIASNNGGKQALETVQRLLPVLCQAHGLTPQQVVAIASNNGGKQALETVQRLLPVLCQAHGLTPEQVVAIASNIGGKQALETVQALLPVLCQAHGLTPQQVVAIASNGGGRPALE

SEQ ID NO: 14 - protein, 530 aa, Artificialsequence
  Repeat-GRex5T1-LPT8-R1
LTPEQVVAIASNIGGKQALETVQALLPVLCQAHGLTPQQVVAIASNGGGKQALETVQRLLPVLCQAHGLTPEQVVAIASHDGGKQALETVQRLLPVLCQAHGLTPEQVVAIASHDGGKQALETVQRLLPVLCQAHGLTPQQVVAIASNGGGKQALETVQRLLPVLCQAHGLTPQQVVAIASNNGGKQALETVQRLLPVLCQAHGLTPEQVVAIASHDGGKQALETVQRLLPVLCQAHGLTPEQVVAIASNIGGKQALETVQALLPVLCQAHGLTPQQVVAIASNGGGKQALETVQRLLPVLCQAHGLTPEQVVAIASNIGGKQALETVQALLPVLCQAHGLTPQQVVAIASNGGGKQALETVQRLLPVLCQAHGLTPEQVVAIASNIGGKQALETVQALLPVLCQAHGLTPEQVVAIASNIGGKQALETVQALLPVLCQAHGLTPEQVVAIASHDGGKQALETVQRLLPVLCQAHGLTPEQVVAIASNIGGKQALETVQALLPVLCQAHGLTPQQVVAIASNGGGRPALE

SEQ ID NO: 15 - protein, 530 aa, Artificialsequence
  Repeat-GRex5T2-L1
LTPEQVVAIASNIGGKQALETVQALLPVLCQAHGLTPQQVVAIASNGGGKQALETVQRLLPVLCQAHGLTPQQVVAIASNNGGKQALETVQRLLPVLCQAHGLTPEQVVAIASNIGGKQALETVQALLPVLCQAHGLTPQQVVAIASNGGGKQALETVQRLLPVLCQAHGLTPEQVVAIASNIGGKQALETVQALLPVLCQAHGLTPQQVVAIASNNGGKQALETVQRLLPVLCQAHGLTPEQVVAIASHDGGKQALETVQRLLPVLCQAHGLTPQQVVAIASNGGGKQALETVQRLLPVLCQAHGLTPEQVVAIASHDGGKQALETVQRLLPVLCQAHGLTPQQVVAIASNGGGKQALETVQRLLPVLCQAHGLTPQQVVAIASNNGGKQALETVQRLLPVLCQAHGLTPQQVVAIASNGGGKQALETVQRLLPVLCQAHGLTPQQVVAIASNGGGKQALETVQRLLPVLCQAHGLTPEQVVAIASHDGGKQALETVQRLLPVLCQAHGLTPQQVVAIASNGGGRPALE

SEQ ID NO: 16 - protein, 530 aa, Artificialsequence
  Repeat-GRex5T2-R1
LTPQQVVAIASNNGGKQALETVQRLLPVLCQAHGLTPEQVVAIASNIGGKQALETVQALLPVLCQAHGLTPQQVVAIASNNGGKQALETVQRLLPVLCQAHGLTPEQVVAIASHDGGKQALETVQRLLPVLCQAHGLTPQQVVAIASNNGGKQALETVQRLLPVLCQAHGLTPQQVVAIASNGGGKQALETVQRLLPVLCQAHGLTPEQVVAIASNIGGKQALETVQALLPVLCQAHGLTPQQVVAIASNNGGKQALETVQRLLPVLCQAHGLTPQQVVAIASNGGGKQALETVQRLLPVLCQAHGLTPEQVVAIASHDGGKQALETVQRLLPVLCQAHGLTPEQVVAIASNIGGKQALETVQALLPVLCQAHGLTPQQVVAIASNGGGKQALETVQRLLPVLCQAHGLTPQQVVAIASNNGGKQALETVQRLLPVLCQAHGLTPEQVVAIASNIGGKQALETVQALLPVLCQAHGLTPQQVVAIASNGGGKQALETVQRLLPVLCQAHGLTPQQVVAIASNGGGRPALE

SEQ ID NO: 17 - protein, 530 aa, Artificialsequence
  Repeat-GRex5T3-L1
LTPQQVVAIASNGGGKQALETVQRLLPVLCQAHGLTPEQVVAIASNIGGKQALETVQALLPVLCQAHGLTPQQVVAIASNGGGKQALETVQRLLPVLCQAHGLTPEQVVAIASNIGGKQALETVQALLPVLCQAHGLTPQQVVAIASNGGGKQALETVQRLLPVLCQAHGLTPQQVVAIASNNGGKQALETVQRLLPVLCQAHGLTPEQVVAIASHDGGKQALETVQRLLPVLCQAHGLTPEQVVAIASNIGGKQALETVQALLPVLCQAHGLTPQQVVAIASNNGGKQALETVQRLLPVLCQAHGLTPQQVVAIASNNGGKQALETVQRLLPVLCQAHGLTPEQVVAIASNIGGKQALETVQALLPVLCQAHGLTPQQVVAIASNGGGKQALETVQRLLPVLCQAHGLTPEQVVAIASNIGGKQALETVQALLPVLCQAHGLTPQQVVAIASNGGGKQALETVQRLLPVLCQAHGLTPQQVVAIASNNGGKQALETVQRLLPVLCQAHGLTPQQVVAIASNGGGRPALE

SEQ ID NO: 18 - protein, 530 aa, Artificialsequence
  Repeat-GRex5T3-R1
LTPQQVVAIASNNGGKQALETVQRLLPVLCQAHGLTPEQVVAIASNIGGKQALETVQALLPVLCQAHGLTPQQVVAIASNGGGKQALETVQRLLPVLCQAHGLTPEQVVAIASHDGGKQALETVQRLLPVLCQAHGLTPEQVVAIASHDGGKQALETVQRLLPVLCQAHGLTPQQVVAIASNGGGKQALETVQRLLPVLCQAHGLTPEQVVAIASHDGGKQALETVQRLLPVLCQAHGLTPEQVVAIASHDGGKQALETVQRLLPVLCQAHGLTPEQVVAIASNIGGKQALETVQALLPVLCQAHGLTPEQVVAIASNIGGKQALETVQALLPVLCQAHGLTPQQVVAIASNNGGKQALETVQRLLPVLCQAHGLTPQQVVAIASNGGGKQALETVQRLLPVLCQAHGLTPQQVVAIASNGGGKQALETVQRLLPVLCQAHGLTPQQVVAIASNNGGKQALETVQRLLPVLCQAHGLTPEQVVAIASNIGGKQALETVQALLPVLCQAHGLTPQQVVAIASNGGGRPALE

SEQ ID NO: 19 - DNA, 2814 bp, Artificialsequence
  GRex2-L TALEN
atgggcgatcctaaaaagaaacgtaaggtcatcgattacccatacgatgttccagattacgctatcgatatcgccgatctacgcacgctcggctacagccagcagcaacaggagaagatcaaaccgaaggttcgttcgacagtggcgcagcaccacgaggcactggtcggccacgggtttacacacgcgcacatcgttgcgttaagccaacacccggcagcgttagggaccgtcgctgtcaagtatcaggacatgatcgcagcgttgccagaggcgacacacgaagcgatcgttggcgtcggcaaacagtggtccggcgcacgcgctctggaggccttgctcacggtggcgggagagttgagaggtccaccgttacagttggacacaggccaacttctcaagattgcaaaacgtggcggcgtgaccgcagtggaggcagtgcatgcatggcgcaatgcactgacgggtgccccgctcaacttgaccccggagcaggtggtggccatcgccagcaatattggtggcaagcaggcgctggagacggtgcaggcgctgttgccggtgctgtgccaggcccacggcttgaccccccagcaggtggtggccatcgccagcaatggcggtggcaagcaggcgctggagacggtccagcggctgttgccggtgctgtgccaggcccacggcttgaccccccagcaggtggtggccatcgccagcaatggcggtggcaagcaggcgctggagacggtccagcggctgttgccggtgctgtgccaggcccacggcttgaccccggagcaggtggtggccatcgccagccacgatggcggcaagcaggcgctggagacggtccagcggctgttgccggtgctgtgccaggcccacggcttgaccccggagcaggtggtggccatcgccagcaatattggtggcaagcaggcgctggagacggtgcaggcgctgttgccggtgctgtgccaggcccacggcttgaccccggagcaggtggtggccatcgccagccacgatggcggcaagcaggcgctggagacggtccagcggctgttgccggtgctgtgccaggcccacggcttgaccccccagcaggtggtggccatcgccagcaatggcggtggcaagcaggcgctggagacggtccagcggctgttgccggtgctgtgccaggcccacggcttgaccccccagcaggtggtggccatcgccagcaataatggtggcaagcaggcgctggagacggtccagcggctgttgccggtgctgtgccaggcccacggcttgaccccggagcaggtggtggccatcgccagcaatattggtggcaagcaggcgctggagacggtgcaggcgctgttgccggtgctgtgccaggcccacggcttgaccccccagcaggtggtggccatcgccagcaatggcggtggcaagcaggcgctggagacggtccagcggctgttgccggtgctgtgccaggcccacggcttgaccccccagcaggtggtggccatcgccagcaataatggtggcaagcaggcgctggagacggtccagcggctgttgccggtgctgtgccaggcccacggcttgaccccccagcaggtggtggccatcgccagcaataatggtggcaagcaggcgctggagacggtccagcggctgttgccggtgctgtgccaggcccacggcttgaccccggagcaggtggtggccatcgccagcaatattggtggcaagcaggcgctggagacggtgcaggcgctgttgccggtgctgtgccaggcccacggcttgaccccggagcaggtggtggccatcgccagccacgatggcggcaagcaggcgctggagacggtccagcggctgttgccggtgctgtgccaggcccacggcttgaccccccagcaggtggtggccatcgccagcaatggcggtggcaagcaggcgctggagacggtccagcggctgttgccggtgctgtgccaggcccacggcttgacccctcagcaggtggtggccatcgccagcaatggcggcggcaggccggcgctggagagcattgttgcccagttatctcgccctgatccggcgttggccgcgttgaccaacgaccacctcgtcgccttggcctgcctcggcgggcgtcctgcgctggatgcagtgaaaaagggattgggggatcctatcagccgttcccagctggtgaagtccgagctggaggagaagaaatccgagttgaggcacaagctgaagtacgtgccccacgagtacatcgagctgatcgagatcgcccggaacagcacccaggaccgtatcctggagatgaaggtgatggagttcttcatgaaggtgtacggctacaggggcaagcacctgggcggctccaggaagcccgacggcgccatctacaccgtgggctcccccatcgactacggcgtgatcgtggacaccaaggcctactccggcggctacaacctgcccatcggccaggccgacgaaatgcagaggtacgtggaggagaaccagaccaggaacaagcacatcaaccccaacgagtggtggaaggtgtacccctccagcgtgaccgagttcaagttcctgttcgtgtccggccacttcaagggcaactacaaggcccagctgaccaggctgaaccacatcaccaactgcaacggcgccgtgctgtccgtggaggagctcctgatcggcggcgagatgatcaaggccggcaccctgaccctggaggaggtgaggaggaagttcaacaacggcgagatcaacttcgcggccgactgataa

SEQ ID NO: 20 - DNA, 2832 bp, Artificialsequence
  GRex2-R TALEN
atgggcgatcctaaaaagaaacgtaaggtcatcgataaggagaccgccgctgccaagttcgagagacagcacatggacagcatcgatatcgccgatctacgcacgctcggctacagccagcagcaacaggagaagatcaaaccgaaggttcgttcgacagtggcgcagcaccacgaggcactggtcggccacgggtttacacacgcgcacatcgttgcgttaagccaacacccggcagcgttagggaccgtcgctgtcaagtatcaggacatgatcgcagcgttgccagaggcgacacacgaagcgatcgttggcgtcggcaaacagtggtccggcgcacgcgctctggaggccttgctcacggtggcgggagagttgagaggtccaccgttacagttggacacaggccaacttctcaagattgcaaaacgtggcggcgtgaccgcagtggaggcagtgcatgcatggcgcaatgcactgacgggtgccccgctcaacttgaccccccagcaggtggtggccatcgccagcaatggcggtggcaagcaggcgctggagacggtccagcggctgttgccggtgctgtgccaggcccacggcttgaccccccagcaggtggtggccatcgccagcaatggcggtggcaagcaggcgctggagacggtccagcggctgttgccggtgctgtgccaggcccacggcttgaccccggagcaggtggtggccatcgccagccacgatggcggcaagcaggcgctggagacggtccagcggctgttgccggtgctgtgccaggcccacggcttgaccccccagcaggtggtggccatcgccagcaatggcggtggcaagcaggcgctggagacggtccagcggctgttgccggtgctgtgccaggcccacggcttgaccccccagcaggtggtggccatcgccagcaatggcggtggcaagcaggcgctggagacggtccagcggctgttgccggtgctgtgccaggcccacggcttgaccccggagcaggtggtggccatcgccagccacgatggcggcaagcaggcgctggagacggtccagcggctgttgccggtgctgtgccaggcccacggcttgaccccccagcaggtggtggccatcgccagcaatggcggtggcaagcaggcgctggagacggtccagcggctgttgccggtgctgtgccaggcccacggcttgaccccggagcaggtggtggccatcgccagccacgatggcggcaagcaggcgctggagacggtccagcggctgttgccggtgctgtgccaggcccacggcttgaccccccagcaggtggtggccatcgccagcaatggcggtggcaagcaggcgctggagacggtccagcggctgttgccggtgctgtgccaggcccacggcttgaccccggagcaggtggtggccatcgccagcaatattggtggcaagcaggcgctggagacggtgcaggcgctgttgccggtgctgtgccaggcccacggcttgaccccggagcaggtggtggccatcgccagccacgatggcggcaagcaggcgctggagacggtccagcggctgttgccggtgctgtgccaggcccacggcttgaccccggagcaggtggtggccatcgccagccacgatggcggcaagcaggcgctggagacggtccagcggctgttgccggtgctgtgccaggcccacggcttgaccccggagcaggtggtggccatcgccagcaatattggtggcaagcaggcgctggagacggtgcaggcgctgttgccggtgctgtgccaggcccacggcttgaccccccagcaggtggtggccatcgccagcaataatggtggcaagcaggcgctggagacggtccagcggctgttgccggtgctgtgccaggcccacggcttgaccccccagcaggtggtggccatcgccagcaataatggtggcaagcaggcgctggagacggtccagcggctgttgccggtgctgtgccaggcccacggcttgacccctcagcaggtggtggccatcgccagcaatggcggcggcaggccggcgctggagagcattgttgcccagttatctcgccctgatccggcgttggccgcgttgaccaacgaccacctcgtcgccttggcctgcctcggcgggcgtcctgcgctggatgcagtgaaaaagggattgggggatcctatcagccgttcccagctggtgaagtccgagctggaggagaagaaatccgagttgaggcacaagctgaagtacgtgccccacgagtacatcgagctgatcgagatcgcccggaacagcacccaggaccgtatcctggagatgaaggtgatggagttcttcatgaaggtgtacggctacaggggcaagcacctgggcggctccaggaagcccgacggcgccatctacaccgtgggctcccccatcgactacggcgtgatcgtggacaccaaggcctactccggcggctacaacctgcccatcggccaggccgacgaaatgcagaggtacgtggaggagaaccagaccaggaacaagcacatcaaccccaacgagtggtggaaggtgtacccctccagcgtgaccgagttcaagttcctgttcgtgtccggccacttcaagggcaactacaaggcccagctgaccaggctgaaccacatcaccaactgcaacggcgccgtgctgtccgtggaggagctcctgatcggcggcgagatgatcaaggccggcaccctgaccctggaggaggtgaggaggaagttcaacaacggcgagatcaacttcgcggccgactgataa

SEQ ID NO: 21 - DNA, 2814 bp, Artificialsequence
  GRex3T2-L TALEN
atgggcgatcctaaaaagaaacgtaaggtcatcgattacccatacgatgttccagattacgctatcgatatcgccgatctacgcacgctcggctacagccagcagcaacaggagaagatcaaaccgaaggttcgttcgacagtggcgcagcaccacgaggcactggtcggccacgggtttacacacgcgcacatcgttgcgttaagccaacacccggcagcgttagggaccgtcgctgtcaagtatcaggacatgatcgcagcgttgccagaggcgacacacgaagcgatcgttggcgtcggcaaacagtggtccggcgcacgcgctctggaggccttgctcacggtggcgggagagttgagaggtccaccgttacagttggacacaggccaacttctcaagattgcaaaacgtggcggcgtgaccgcagtggaggcagtgcatgcatggcgcaatgcactgacgggtgccccgctcaacttgaccccccagcaggtggtggccatcgccagcaataatggtggcaagcaggcgctggagacggtccagcggctgttgccggtgctgtgccaggcccacggcttgaccccggagcaggtggtggccatcgccagccacgatggcggcaagcaggcgctggagacggtccagcggctgttgccggtgctgtgccaggcccacggcttgaccccggagcaggtggtggccatcgccagccacgatggcggcaagcaggcgctggagacggtccagcggctgttgccggtgctgtgccaggcccacggcttgaccccccagcaggtggtggccatcgccagcaatggcggtggcaagcaggcgctggagacggtccagcggctgttgccggtgctgtgccaggcccacggcttgaccccccagcaggtggtggccatcgccagcaataatggtggcaagcaggcgctggagacggtccagcggctgttgccggtgctgtgccaggcccacggcttgaccccccagcaggtggtggccatcgccagcaataatggtggcaagcaggcgctggagacggtccagcggctgttgccggtgctgtgccaggcccacggcttgaccccccagcaggtggtggccatcgccagcaatggcggtggcaagcaggcgctggagacggtccagcggctgttgccggtgctgtgccaggcccacggcttgaccccccagcaggtggtggccatcgccagcaataatggtggcaagcaggcgctggagacggtccagcggctgttgccggtgctgtgccaggcccacggcttgaccccccagcaggtggtggccatcgccagcaatggcggtggcaagcaggcgctggagacggtccagcggctgttgccggtgctgtgccaggcccacggcttgaccccccagcaggtggtggccatcgccagcaataatggtggcaagcaggcgctggagacggtccagcggctgttgccggtgctgtgccaggcccacggcttgaccccggagcaggtggtggccatcgccagccacgatggcggcaagcaggcgctggagacggtccagcggctgttgccggtgctgtgccaggcccacggcttgaccccccagcaggtggtggccatcgccagcaatggcggtggcaagcaggcgctggagacggtccagcggctgttgccggtgctgtgccaggcccacggcttgaccccggagcaggtggtggccatcgccagccacgatggcggcaagcaggcgctggagacggtccagcggctgttgccggtgctgtgccaggcccacggcttgaccccccagcaggtggtggccatcgccagcaatggcggtggcaagcaggcgctggagacggtccagcggctgttgccggtgctgtgccaggcccacggcttgaccccccagcaggtggtggccatcgccagcaataatggtggcaagcaggcgctggagacggtccagcggctgttgccggtgctgtgccaggcccacggcttgacccctcagcaggtggtggccatcgccagcaatggcggcggcaggccggcgctggagagcattgttgcccagttatctcgccctgatccggcgttggccgcgttgaccaacgaccacctcgtcgccttggcctgcctcggcgggcgtcctgcgctggatgcagtgaaaaagggattgggggatcctatcagccgttcccagctggtgaagtccgagctggaggagaagaaatccgagttgaggcacaagctgaagtacgtgccccacgagtacatcgagctgatcgagatcgcccggaacagcacccaggaccgtatcctggagatgaaggtgatggagttcttcatgaaggtgtacggctacaggggcaagcacctgggcggctccaggaagcccgacggcgccatctacaccgtgggctcccccatcgactacggcgtgatcgtggacaccaaggcctactccggcggctacaacctgcccatcggccaggccgacgaaatgcagaggtacgtggaggagaaccagaccaggaacaagcacatcaaccccaacgagtggtggaaggtgtacccctccagcgtgaccgagttcaagttcctgttcgtgtccggccacttcaagggcaactacaaggcccagctgaccaggctgaaccacatcaccaactgcaacggcgccgtgctgtccgtggaggagctcctgatcggcggcgagatgatcaaggccggcaccctgaccctggaggaggtgaggaggaagttcaacaacggcgagatcaacttcgcggccgactgataa

SEQ ID NO: 22 - DNA, 2832 bp, Artificialsequence
  GRex3T2-R TALEN
atgggcgatcctaaaaagaaacgtaaggtcatcgataaggagaccgccgctgccaagttcgagagacagcacatggacagcatcgatatcgccgatctacgcacgctcggctacagccagcagcaacaggagaagatcaaaccgaaggttcgttcgacagtggcgcagcaccacgaggcactggtcggccacgggtttacacacgcgcacatcgttgcgttaagccaacacccggcagcgttagggaccgtcgctgtcaagtatcaggacatgatcgcagcgttgccagaggcgacacacgaagcgatcgttggcgtcggcaaacagtggtccggcgcacgcgctctggaggccttgctcacggtggcgggagagttgagaggtccaccgttacagttggacacaggccaacttctcaagattgcaaaacgtggcggcgtgaccgcagtggaggcagtgcatgcatggcgcaatgcactgacgggtgccccgctcaacttgaccccccagcaggtggtggccatcgccagcaatggcggtggcaagcaggcgctggagacggtccagcggctgttgccggtgctgtgccaggcccacggcttgaccccggagcaggtggtggccatcgccagcaatattggtggcaagcaggcgctggagacggtgcaggcgctgttgccggtgctgtgccaggcccacggcttgaccccggagcaggtggtggccatcgccagcaatattggtggcaagcaggcgctggagacggtgcaggcgctgttgccggtgctgtgccaggcccacggcttgaccccccagcaggtggtggccatcgccagcaataatggtggcaagcaggcgctggagacggtccagcggctgttgccggtgctgtgccaggcccacggcttgaccccggagcaggtggtggccatcgccagcaatattggtggcaagcaggcgctggagacggtgcaggcgctgttgccggtgctgtgccaggcccacggcttgaccccggagcaggtggtggccatcgccagccacgatggcggcaagcaggcgctggagacggtccagcggctgttgccggtgctgtgccaggcccacggcttgaccccccagcaggtggtggccatcgccagcaatggcggtggcaagcaggcgctggagacggtccagcggctgttgccggtgctgtgccaggcccacggcttgaccccggagcaggtggtggccatcgccagccacgatggcggcaagcaggcgctggagacggtccagcggctgttgccggtgctgtgccaggcccacggcttgaccccggagcaggtggtggccatcgccagccacgatggcggcaagcaggcgctggagacggtccagcggctgttgccggtgctgtgccaggcccacggcttgaccccggagcaggtggtggccatcgccagcaatattggtggcaagcaggcgctggagacggtgcaggcgctgttgccggtgctgtgccaggcccacggcttgaccccccagcaggtggtggccatcgccagcaatggcggtggcaagcaggcgctggagacggtccagcggctgttgccggtgctgtgccaggcccacggcttgaccccggagcaggtggtggccatcgccagcaatattggtggcaagcaggcgctggagacggtgcaggcgctgttgccggtgctgtgccaggcccacggcttgaccccggagcaggtggtggccatcgccagcaatattggtggcaagcaggcgctggagacggtgcaggcgctgttgccggtgctgtgccaggcccacggcttgaccccccagcaggtggtggccatcgccagcaatggcggtggcaagcaggcgctggagacggtccagcggctgttgccggtgctgtgccaggcccacggcttgaccccccagcaggtggtggccatcgccagcaataatggtggcaagcaggcgctggagacggtccagcggctgttgccggtgctgtgccaggcccacggcttgacccctcagcaggtggtggccatcgccagcaatggcggcggcaggccggcgctggagagcattgttgcccagttatctcgccctgatccggcgttggccgcgttgaccaacgaccacctcgtcgccttggcctgcctcggcgggcgtcctgcgctggatgcagtgaaaaagggattgggggatcctatcagccgttcccagctggtgaagtccgagctggaggagaagaaatccgagttgaggcacaagctgaagtacgtgccccacgagtacatcgagctgatcgagatcgcccggaacagcacccaggaccgtatcctggagatgaaggtgatggagttcttcatgaaggtgtacggctacaggggcaagcacctgggcggctccaggaagcccgacggcgccatctacaccgtgggctcccccatcgactacggcgtgatcgtggacaccaaggcctactccggcggctacaacctgcccatcggccaggccgacgaaatgcagaggtacgtggaggagaaccagaccaggaacaagcacatcaaccccaacgagtggtggaaggtgtacccctccagcgtgaccgagttcaagttcctgttcgtgtccggccacttcaagggcaactacaaggcccagctgaccaggctgaaccacatcaccaactgcaacggcgccgtgctgtccgtggaggagctcctgatcggcggcgagatgatcaaggccggcaccctgaccctggaggaggtgaggaggaagttcaacaacggcgagatcaacttcgcggccgactgataa

SEQ ID NO: 23 - DNA, 2814 bp, Artificialsequence
  GRex3T4-L TALEN
atgggcgatcctaaaaagaaacgtaaggtcatcgattacccatacgatgttccagattacgctatcgatatcgccgatctacgcacgctcggctacagccagcagcaacaggagaagatcaaaccgaaggttcgttcgacagtggcgcagcaccacgaggcactggtcggccacgggtttacacacgcgcacatcgttgcgttaagccaacacccggcagcgttagggaccgtcgctgtcaagtatcaggacatgatcgcagcgttgccagaggcgacacacgaagcgatcgttggcgtcggcaaacagtggtccggcgcacgcgctctggaggccttgctcacggtggcgggagagttgagaggtccaccgttacagttggacacaggccaacttctcaagattgcaaaacgtggcggcgtgaccgcagtggaggcagtgcatgcatggcgcaatgcactgacgggtgccccgctcaacttgaccccccagcaggtggtggccatcgccagcaataatggtggcaagcaggcgctggagacggtccagcggctgttgccggtgctgtgccaggcccacggcttgaccccggagcaggtggtggccatcgccagccacgatggcggcaagcaggcgctggagacggtccagcggctgttgccggtgctgtgccaggcccacggcttgaccccccagcaggtggtggccatcgccagcaatggcggtggcaagcaggcgctggagacggtccagcggctgttgccggtgctgtgccaggcccacggcttgaccccggagcaggtggtggccatcgccagccacgatggcggcaagcaggcgctggagacggtccagcggctgttgccggtgctgtgccaggcccacggcttgaccccccagcaggtggtggccatcgccagcaatggcggtggcaagcaggcgctggagacggtccagcggctgttgccggtgctgtgccaggcccacggcttgaccccccagcaggtggtggccatcgccagcaataatggtggcaagcaggcgctggagacggtccagcggctgttgccggtgctgtgccaggcccacggcttgaccccggagcaggtggtggccatcgccagcaatattggtggcaagcaggcgctggagacggtgcaggcgctgttgccggtgctgtgccaggcccacggcttgaccccccagcaggtggtggccatcgccagcaatggcggtggcaagcaggcgctggagacggtccagcggctgttgccggtgctgtgccaggcccacggcttgaccccccagcaggtggtggccatcgccagcaataatggtggcaagcaggcgctggagacggtccagcggctgttgccggtgctgtgccaggcccacggcttgaccccggagcaggtggtggccatcgccagcaatattggtggcaagcaggcgctggagacggtgcaggcgctgttgccggtgctgtgccaggcccacggcttgaccccggagcaggtggtggccatcgccagcaatattggtggcaagcaggcgctggagacggtgcaggcgctgttgccggtgctgtgccaggcccacggcttgaccccccagcaggtggtggccatcgccagcaataatggtggcaagcaggcgctggagacggtccagcggctgttgccggtgctgtgccaggcccacggcttgaccccggagcaggtggtggccatcgccagccacgatggcggcaagcaggcgctggagacggtccagcggctgttgccggtgctgtgccaggcccacggcttgaccccccagcaggtggtggccatcgccagcaatggcggtggcaagcaggcgctggagacggtccagcggctgttgccggtgctgtgccaggcccacggcttgaccccccagcaggtggtggccatcgccagcaatggcggtggcaagcaggcgctggagacggtccagcggctgttgccggtgctgtgccaggcccacggcttgacccctcagcaggtggtggccatcgccagcaatggcggcggcaggccggcgctggagagcattgttgcccagttatctcgccctgatccggcgttggccgcgttgaccaacgaccacctcgtcgccttggcctgcctcggcgggcgtcctgcgctggatgcagtgaaaaagggattgggggatcctatcagccgttcccagctggtgaagtccgagctggaggagaagaaatccgagttgaggcacaagctgaagtacgtgccccacgagtacatcgagctgatcgagatcgcccggaacagcacccaggaccgtatcctggagatgaaggtgatggagttcttcatgaaggtgtacggctacaggggcaagcacctgggcggctccaggaagcccgacggcgccatctacaccgtgggctcccccatcgactacggcgtgatcgtggacaccaaggcctactccggcggctacaacctgcccatcggccaggccgacgaaatgcagaggtacgtggaggagaaccagaccaggaacaagcacatcaaccccaacgagtggtggaaggtgtacccctccagcgtgaccgagttcaagttcctgttcgtgtccggccacttcaagggcaactacaaggcccagctgaccaggctgaaccacatcaccaactgcaacggcgccgtgctgtccgtggaggagctcctgatcggcggcgagatgatcaaggccggcaccctgaccctggaggaggtgaggaggaagttcaacaacggcgagatcaacttcgcggccgactgataa

SEQ ID NO: 24 - DNA, 2832 bp, Artificialsequence
  GRex3T4-R TALEN
atgggcgatcctaaaaagaaacgtaaggtcatcgataaggagaccgccgctgccaagttcgagagacagcacatggacagcatcgatatcgccgatctacgcacgctcggctacagccagcagcaacaggagaagatcaaaccgaaggttcgttcgacagtggcgcagcaccacgaggcactggtcggccacgggtttacacacgcgcacatcgttgcgttaagccaacacccggcagcgttagggaccgtcgctgtcaagtatcaggacatgatcgcagcgttgccagaggcgacacacgaagcgatcgttggcgtcggcaaacagtggtccggcgcacgcgctctggaggccttgctcacggtggcgggagagttgagaggtccaccgttacagttggacacaggccaacttctcaagattgcaaaacgtggcggcgtgaccgcagtggaggcagtgcatgcatggcgcaatgcactgacgggtgccccgctcaacttgaccccccagcaggtggtggccatcgccagcaatggcggtggcaagcaggcgctggagacggtccagcggctgttgccggtgctgtgccaggcccacggcttgaccccggagcaggtggtggccatcgccagccacgatggcggcaagcaggcgctggagacggtccagcggctgttgccggtgctgtgccaggcccacggcttgaccccggagcaggtggtggccatcgccagccacgatggcggcaagcaggcgctggagacggtccagcggctgttgccggtgctgtgccaggcccacggcttgaccccggagcaggtggtggccatcgccagcaatattggtggcaagcaggcgctggagacggtgcaggcgctgttgccggtgctgtgccaggcccacggcttgaccccggagcaggtggtggccatcgccagccacgatggcggcaagcaggcgctggagacggtccagcggctgttgccggtgctgtgccaggcccacggcttgaccccggagcaggtggtggccatcgccagcaatattggtggcaagcaggcgctggagacggtgcaggcgctgttgccggtgctgtgccaggcccacggcttgaccccggagcaggtggtggccatcgccagcaatattggtggcaagcaggcgctggagacggtgcaggcgctgttgccggtgctgtgccaggcccacggcttgaccccccagcaggtggtggccatcgccagcaataatggtggcaagcaggcgctggagacggtccagcggctgttgccggtgctgtgccaggcccacggcttgaccccccagcaggtggtggccatcgccagcaatggcggtggcaagcaggcgctggagacggtccagcggctgttgccggtgctgtgccaggcccacggcttgaccccccagcaggtggtggccatcgccagcaatggcggtggcaagcaggcgctggagacggtccagcggctgttgccggtgctgtgccaggcccacggcttgaccccggagcaggtggtggccatcgccagcaatattggtggcaagcaggcgctggagacggtgcaggcgctgttgccggtgctgtgccaggcccacggcttgaccccggagcaggtggtggccatcgccagcaatattggtggcaagcaggcgctggagacggtgcaggcgctgttgccggtgctgtgccaggcccacggcttgaccccccagcaggtggtggccatcgccagcaataatggtggcaagcaggcgctggagacggtccagcggctgttgccggtgctgtgccaggcccacggcttgaccccggagcaggtggtggccatcgccagcaatattggtggcaagcaggcgctggagacggtgcaggcgctgttgccggtgctgtgccaggcccacggcttgaccccggagcaggtggtggccatcgccagccacgatggcggcaagcaggcgctggagacggtccagcggctgttgccggtgctgtgccaggcccacggcttgacccctcagcaggtggtggccatcgccagcaatggcggcggcaggccggcgctggagagcattgttgcccagttatctcgccctgatccggcgttggccgcgttgaccaacgaccacctcgtcgccttggcctgcctcggcgggcgtcctgcgctggatgcagtgaaaaagggattgggggatcctatcagccgttcccagctggtgaagtccgagctggaggagaagaaatccgagttgaggcacaagctgaagtacgtgccccacgagtacatcgagctgatcgagatcgcccggaacagcacccaggaccgtatcctggagatgaaggtgatggagttcttcatgaaggtgtacggctacaggggcaagcacctgggcggctccaggaagcccgacggcgccatctacaccgtgggctcccccatcgactacggcgtgatcgtggacaccaaggcctactccggcggctacaacctgcccatcggccaggccgacgaaatgcagaggtacgtggaggagaaccagaccaggaacaagcacatcaaccccaacgagtggtggaaggtgtacccctccagcgtgaccgagttcaagttcctgttcgtgtccggccacttcaagggcaactacaaggcccagctgaccaggctgaaccacatcaccaactgcaacggcgccgtgctgtccgtggaggagctcctgatcggcggcgagatgatcaaggccggcaccctgaccctggaggaggtgaggaggaagttcaacaacggcgagatcaacttcgcggccgactgataa

SEQ ID NO: 25 - DNA, 2814 bp, Artificialsequence
  GRex5T1-L TALEN
atgggcgatcctaaaaagaaacgtaaggtcatcgattacccatacgatgttccagattacgctatcgatatcgccgatctacgcacgctcggctacagccagcagcaacaggagaagatcaaaccgaaggttcgttcgacagtggcgcagcaccacgaggcactggtcggccacgggtttacacacgcgcacatcgttgcgttaagccaacacccggcagcgttagggaccgtcgctgtcaagtatcaggacatgatcgcagcgttgccagaggcgacacacgaagcgatcgttggcgtcggcaaacagtggtccggcgcacgcgctctggaggccttgctcacggtggcgggagagttgagaggtccaccgttacagttggacacaggccaacttctcaagattgcaaaacgtggcggcgtgaccgcagtggaggcagtgcatgcatggcgcaatgcactgacgggtgccccgctcaacttgaccccccagcaggtggtggccatcgccagcaataatggtggcaagcaggcgctggagacggtccagcggctgttgccggtgctgtgccaggcccacggcttgaccccccagcaggtggtggccatcgccagcaataatggtggcaagcaggcgctggagacggtccagcggctgttgccggtgctgtgccaggcccacggcttgaccccccagcaggtggtggccatcgccagcaatggcggtggcaagcaggcgctggagacggtccagcggctgttgccggtgctgtgccaggcccacggcttgaccccccagcaggtggtggccatcgccagcaataatggtggcaagcaggcgctggagacggtccagcggctgttgccggtgctgtgccaggcccacggcttgaccccccagcaggtggtggccatcgccagcaatggcggtggcaagcaggcgctggagacggtccagcggctgttgccggtgctgtgccaggcccacggcttgaccccggagcaggtggtggccatcgccagccacgatggcggcaagcaggcgctggagacggtccagcggctgttgccggtgctgtgccaggcccacggcttgaccccggagcaggtggtggccatcgccagcaatattggtggcaagcaggcgctggagacggtgcaggcgctgttgccggtgctgtgccaggcccacggcttgaccccggagcaggtggtggccatcgccagccacgatggcggcaagcaggcgctggagacggtccagcggctgttgccggtgctgtgccaggcccacggcttgaccccccagcaggtggtggccatcgccagcaatggcggtggcaagcaggcgctggagacggtccagcggctgttgccggtgctgtgccaggcccacggcttgaccccccagcaggtggtggccatcgccagcaataatggtggcaagcaggcgctggagacggtccagcggctgttgccggtgctgtgccaggcccacggcttgaccccccagcaggtggtggccatcgccagcaatggcggtggcaagcaggcgctggagacggtccagcggctgttgccggtgctgtgccaggcccacggcttgaccccccagcaggtggtggccatcgccagcaatggcggtggcaagcaggcgctggagacggtccagcggctgttgccggtgctgtgccaggcccacggcttgaccccccagcaggtggtggccatcgccagcaataatggtggcaagcaggcgctggagacggtccagcggctgttgccggtgctgtgccaggcccacggcttgaccccccagcaggtggtggccatcgccagcaataatggtggcaagcaggcgctggagacggtccagcggctgttgccggtgctgtgccaggcccacggcttgaccccggagcaggtggtggccatcgccagcaatattggtggcaagcaggcgctggagacggtgcaggcgctgttgccggtgctgtgccaggcccacggcttgacccctcagcaggtggtggccatcgccagcaatggcggcggcaggccggcgctggagagcattgttgcccagttatctcgccctgatccggcgttggccgcgttgaccaacgaccacctcgtcgccttggcctgcctcggcgggcgtcctgcgctggatgcagtgaaaaagggattgggggatcctatcagccgttcccagctggtgaagtccgagctggaggagaagaaatccgagttgaggcacaagctgaagtacgtgccccacgagtacatcgagctgatcgagatcgcccggaacagcacccaggaccgtatcctggagatgaaggtgatggagttcttcatgaaggtgtacggctacaggggcaagcacctgggcggctccaggaagcccgacggcgccatctacaccgtgggctcccccatcgactacggcgtgatcgtggacaccaaggcctactccggcggctacaacctgcccatcggccaggccgacgaaatgcagaggtacgtggaggagaaccagaccaggaacaagcacatcaaccccaacgagtggtggaaggtgtacccctccagcgtgaccgagttcaagttcctgttcgtgtccggccacttcaagggcaactacaaggcccagctgaccaggctgaaccacatcaccaactgcaacggcgccgtgctgtccgtggaggagctcctgatcggcggcgagatgatcaaggccggcaccctgaccctggaggaggtgaggaggaagttcaacaacggcgagatcaacttcgcggccgactgataa

SEQ ID NO: 26 - DNA, 2832 bp, Artificialsequence
  GRex5T1-R TALEN
atgggcgatcctaaaaagaaacgtaaggtcatcgataaggagaccgccgctgccaagttcgagagacagcacatggacagcatcgatatcgccgatctacgcacgctcggctacagccagcagcaacaggagaagatcaaaccgaaggttcgttcgacagtggcgcagcaccacgaggcactggtcggccacgggtttacacacgcgcacatcgttgcgttaagccaacacccggcagcgttagggaccgtcgctgtcaagtatcaggacatgatcgcagcgttgccagaggcgacacacgaagcgatcgttggcgtcggcaaacagtggtccggcgcacgcgctctggaggccttgctcacggtggcgggagagttgagaggtccaccgttacagttggacacaggccaacttctcaagattgcaaaacgtggcggcgtgaccgcagtggaggcagtgcatgcatggcgcaatgcactgacgggtgccccgctcaacttgaccccggagcaggtggtggccatcgccagcaatattggtggcaagcaggcgctggagacggtgcaggcgctgttgccggtgctgtgccaggcccacggcttgaccccccagcaggtggtggccatcgccagcaatggcggtggcaagcaggcgctggagacggtccagcggctgttgccggtgctgtgccaggcccacggcttgaccccggagcaggtggtggccatcgccagccacgatggcggcaagcaggcgctggagacggtccagcggctgttgccggtgctgtgccaggcccacggcttgaccccggagcaggtggtggccatcgccagccacgatggcggcaagcaggcgctggagacggtccagcggctgttgccggtgctgtgccaggcccacggcttgaccccccagcaggtggtggccatcgccagcaatggcggtggcaagcaggcgctggagacggtccagcggctgttgccggtgctgtgccaggcccacggcttgaccccccagcaggtggtggccatcgccagcaataatggtggcaagcaggcgctggagacggtccagcggctgttgccggtgctgtgccaggcccacggcttgaccccggagcaggtggtggccatcgccagccacgatggcggcaagcaggcgctggagacggtccagcggctgttgccggtgctgtgccaggcccacggcttgaccccggagcaggtggtggccatcgccagcaatattggtggcaagcaggcgctggagacggtgcaggcgctgttgccggtgctgtgccaggcccacggcttgaccccccagcaggtggtggccatcgccagcaatggcggtggcaagcaggcgctggagacggtccagcggctgttgccggtgctgtgccaggcccacggcttgaccccggagcaggtggtggccatcgccagcaatattggtggcaagcaggcgctggagacggtgcaggcgctgttgccggtgctgtgccaggcccacggcttgaccccccagcaggtggtggccatcgccagcaatggcggtggcaagcaggcgctggagacggtccagcggctgttgccggtgctgtgccaggcccacggcttgaccccggagcaggtggtggccatcgccagcaatattggtggcaagcaggcgctggagacggtgcaggcgctgttgccggtgctgtgccaggcccacggcttgaccccggagcaggtggtggccatcgccagcaatattggtggcaagcaggcgctggagacggtgcaggcgctgttgccggtgctgtgccaggcccacggcttgaccccggagcaggtggtggccatcgccagccacgatggcggcaagcaggcgctggagacggtccagcggctgttgccggtgctgtgccaggcccacggcttgaccccggagcaggtggtggccatcgccagcaatattggtggcaagcaggcgctggagacggtgcaggcgctgttgccggtgctgtgccaggcccacggcttgacccctcagcaggtggtggccatcgccagcaatggcggcggcaggccggcgctggagagcattgttgcccagttatctcgccctgatccggcgttggccgcgttgaccaacgaccacctcgtcgccttggcctgcctcggcgggcgtcctgcgctggatgcagtgaaaaagggattgggggatcctatcagccgttcccagctggtgaagtccgagctggaggagaagaaatccgagttgaggcacaagctgaagtacgtgccccacgagtacatcgagctgatcgagatcgcccggaacagcacccaggaccgtatcctggagatgaaggtgatggagttcttcatgaaggtgtacggctacaggggcaagcacctgggcggctccaggaagcccgacggcgccatctacaccgtgggctcccccatcgactacggcgtgatcgtggacaccaaggcctactccggcggctacaacctgcccatcggccaggccgacgaaatgcagaggtacgtggaggagaaccagaccaggaacaagcacatcaaccccaacgagtggtggaaggtgtacccctccagcgtgaccgagttcaagttcctgttcgtgtccggccacttcaagggcaactacaaggcccagctgaccaggctgaaccacatcaccaactgcaacggcgccgtgctgtccgtggaggagctcctgatcggcggcgagatgatcaaggccggcaccctgaccctggaggaggtgaggaggaagttcaacaacggcgagatcaacttcgcggccgactgataa

SEQ ID NO: 27 - DNA, 2814 bp, Artificialsequence
  GRex5T2-L TALEN
atgggcgatcctaaaaagaaacgtaaggtcatcgattacccatacgatgttccagattacgctatcgatatcgccgatctacgcacgctcggctacagccagcagcaacaggagaagatcaaaccgaaggttcgttcgacagtggcgcagcaccacgaggcactggtcggccacgggtttacacacgcgcacatcgttgcgttaagccaacacccggcagcgttagggaccgtcgctgtcaagtatcaggacatgatcgcagcgttgccagaggcgacacacgaagcgatcgttggcgtcggcaaacagtggtccggcgcacgcgctctggaggccttgctcacggtggcgggagagttgagaggtccaccgttacagttggacacaggccaacttctcaagattgcaaaacgtggcggcgtgaccgcagtggaggcagtgcatgcatggcgcaatgcactgacgggtgccccgctcaacttgaccccggagcaggtggtggccatcgccagcaatattggtggcaagcaggcgctggagacggtgcaggcgctgttgccggtgctgtgccaggcccacggcttgaccccccagcaggtggtggccatcgccagcaatggcggtggcaagcaggcgctggagacggtccagcggctgttgccggtgctgtgccaggcccacggcttgaccccccagcaggtggtggccatcgccagcaataatggtggcaagcaggcgctggagacggtccagcggctgttgccggtgctgtgccaggcccacggcttgaccccggagcaggtggtggccatcgccagcaatattggtggcaagcaggcgctggagacggtgcaggcgctgttgccggtgctgtgccaggcccacggcttgaccccccagcaggtggtggccatcgccagcaatggcggtggcaagcaggcgctggagacggtccagcggctgttgccggtgctgtgccaggcccacggcttgaccccggagcaggtggtggccatcgccagcaatattggtggcaagcaggcgctggagacggtgcaggcgctgttgccggtgctgtgccaggcccacggcttgaccccccagcaggtggtggccatcgccagcaataatggtggcaagcaggcgctggagacggtccagcggctgttgccggtgctgtgccaggcccacggcttgaccccggagcaggtggtggccatcgccagccacgatggcggcaagcaggcgctggagacggtccagcggctgttgccggtgctgtgccaggcccacggcttgaccccccagcaggtggtggccatcgccagcaatggcggtggcaagcaggcgctggagacggtccagcggctgttgccggtgctgtgccaggcccacggcttgaccccggagcaggtggtggccatcgccagccacgatggcggcaagcaggcgctggagacggtccagcggctgttgccggtgctgtgccaggcccacggcttgaccccccagcaggtggtggccatcgccagcaatggcggtggcaagcaggcgctggagacggtccagcggctgttgccggtgctgtgccaggcccacggcttgaccccccagcaggtggtggccatcgccagcaataatggtggcaagcaggcgctggagacggtccagcggctgttgccggtgctgtgccaggcccacggcttgaccccccagcaggtggtggccatcgccagcaatggcggtggcaagcaggcgctggagacggtccagcggctgttgccggtgctgtgccaggcccacggcttgaccccccagcaggtggtggccatcgccagcaatggcggtggcaagcaggcgctggagacggtccagcggctgttgccggtgctgtgccaggcccacggcttgaccccggagcaggtggtggccatcgccagccacgatggcggcaagcaggcgctggagacggtccagcggctgttgccggtgctgtgccaggcccacggcttgacccctcagcaggtggtggccatcgccagcaatggcggcggcaggccggcgctggagagcattgttgcccagttatctcgccctgatccggcgttggccgcgttgaccaacgaccacctcgtcgccttggcctgcctcggcgggcgtcctgcgctggatgcagtgaaaaagggattgggggatcctatcagccgttcccagctggtgaagtccgagctggaggagaagaaatccgagttgaggcacaagctgaagtacgtgccccacgagtacatcgagctgatcgagatcgcccggaacagcacccaggaccgtatcctggagatgaaggtgatggagttcttcatgaaggtgtacggctacaggggcaagcacctgggcggctccaggaagcccgacggcgccatctacaccgtgggctcccccatcgactacggcgtgatcgtggacaccaaggcctactccggcggctacaacctgcccatcggccaggccgacgaaatgcagaggtacgtggaggagaaccagaccaggaacaagcacatcaaccccaacgagtggtggaaggtgtacccctccagcgtgaccgagttcaagttcctgttcgtgtccggccacttcaagggcaactacaaggcccagctgaccaggctgaaccacatcaccaactgcaacggcgccgtgctgtccgtggaggagctcctgatcggcggcgagatgatcaaggccggcaccctgaccctggaggaggtgaggaggaagttcaacaacggcgagatcaacttcgcggccgactgataa

SEQ ID NO: 28 - DNA, 2832 bp, Artificialsequence
  GRex5T2-R TALEN
atgggcgatcctaaaaagaaacgtaaggtcatcgataaggagaccgccgctgccaagttcgagagacagcacatggacagcatcgatatcgccgatctacgcacgctcggctacagccagcagcaacaggagaagatcaaaccgaaggttcgttcgacagtggcgcagcaccacgaggcactggtcggccacgggtttacacacgcgcacatcgttgcgttaagccaacacccggcagcgttagggaccgtcgctgtcaagtatcaggacatgatcgcagcgttgccagaggcgacacacgaagcgatcgttggcgtcggcaaacagtggtccggcgcacgcgctctggaggccttgctcacggtggcgggagagttgagaggtccaccgttacagttggacacaggccaacttctcaagattgcaaaacgtggcggcgtgaccgcagtggaggcagtgcatgcatggcgcaatgcactgacgggtgccccgctcaacttgaccccccagcaggtggtggccatcgccagcaataatggtggcaagcaggcgctggagacggtccagcggctgttgccggtgctgtgccaggcccacggcttgaccccggagcaggtggtggccatcgccagcaatattggtggcaagcaggcgctggagacggtgcaggcgctgttgccggtgctgtgccaggcccacggcttgaccccccagcaggtggtggccatcgccagcaataatggtggcaagcaggcgctggagacggtccagcggctgttgccggtgctgtgccaggcccacggcttgaccccggagcaggtggtggccatcgccagccacgatggcggcaagcaggcgctggagacggtccagcggctgttgccggtgctgtgccaggcccacggcttgaccccccagcaggtggtggccatcgccagcaataatggtggcaagcaggcgctggagacggtccagcggctgttgccggtgctgtgccaggcccacggcttgaccccccagcaggtggtggccatcgccagcaatggcggtggcaagcaggcgctggagacggtccagcggctgttgccggtgctgtgccaggcccacggcttgaccccggagcaggtggtggccatcgccagcaatattggtggcaagcaggcgctggagacggtgcaggcgctgttgccggtgctgtgccaggcccacggcttgaccccccagcaggtggtggccatcgccagcaataatggtggcaagcaggcgctggagacggtccagcggctgttgccggtgctgtgccaggcccacggcttgaccccccagcaggtggtggccatcgccagcaatggcggtggcaagcaggcgctggagacggtccagcggctgttgccggtgctgtgccaggcccacggcttgaccccggagcaggtggtggccatcgccagccacgatggcggcaagcaggcgctggagacggtccagcggctgttgccggtgctgtgccaggcccacggcttgaccccggagcaggtggtggccatcgccagcaatattggtggcaagcaggcgctggagacggtgcaggcgctgttgccggtgctgtgccaggcccacggcttgaccccccagcaggtggtggccatcgccagcaatggcggtggcaagcaggcgctggagacggtccagcggctgttgccggtgctgtgccaggcccacggcttgaccccccagcaggtggtggccatcgccagcaataatggtggcaagcaggcgctggagacggtccagcggctgttgccggtgctgtgccaggcccacggcttgaccccggagcaggtggtggccatcgccagcaatattggtggcaagcaggcgctggagacggtgcaggcgctgttgccggtgctgtgccaggcccacggcttgaccccccagcaggtggtggccatcgccagcaatggcggtggcaagcaggcgctggagacggtccagcggctgttgccggtgctgtgccaggcccacggcttgacccctcagcaggtggtggccatcgccagcaatggcggcggcaggccggcgctggagagcattgttgcccagttatctcgccctgatccggcgttggccgcgttgaccaacgaccacctcgtcgccttggcctgcctcggcgggcgtcctgcgctggatgcagtgaaaaagggattgggggatcctatcagccgttcccagctggtgaagtccgagctggaggagaagaaatccgagttgaggcacaagctgaagtacgtgccccacgagtacatcgagctgatcgagatcgcccggaacagcacccaggaccgtatcctggagatgaaggtgatggagttcttcatgaaggtgtacggctacaggggcaagcacctgggcggctccaggaagcccgacggcgccatctacaccgtgggctcccccatcgactacggcgtgatcgtggacaccaaggcctactccggcggctacaacctgcccatcggccaggccgacgaaatgcagaggtacgtggaggagaaccagaccaggaacaagcacatcaaccccaacgagtggtggaaggtgtacccctccagcgtgaccgagttcaagttcctgttcgtgtccggccacttcaagggcaactacaaggcccagctgaccaggctgaaccacatcaccaactgcaacggcgccgtgctgtccgtggaggagctcctgatcggcggcgagatgatcaaggccggcaccctgaccctggaggaggtgaggaggaagttcaacaacggcgagatcaacttcgcggccgactgataa

SEQ ID NO: 29 - DNA, 2814 bp, Artificialsequence
  GRex5T3-L TALEN
atgggcgatcctaaaaagaaacgtaaggtcatcgattacccatacgatgttccagattacgctatcgatatcgccgatctacgcacgctcggctacagccagcagcaacaggagaagatcaaaccgaaggttcgttcgacagtggcgcagcaccacgaggcactggtcggccacgggtttacacacgcgcacatcgttgcgttaagccaacacccggcagcgttagggaccgtcgctgtcaagtatcaggacatgatcgcagcgttgccagaggcgacacacgaagcgatcgttggcgtcggcaaacagtggtccggcgcacgcgctctggaggccttgctcacggtggcgggagagttgagaggtccaccgttacagttggacacaggccaacttctcaagattgcaaaacgtggcggcgtgaccgcagtggaggcagtgcatgcatggcgcaatgcactgacgggtgccccgctcaacttgaccccccagcaggtggtggccatcgccagcaatggcggtggcaagcaggcgctggagacggtccagcggctgttgccggtgctgtgccaggcccacggcttgaccccggagcaggtggtggccatcgccagcaatattggtggcaagcaggcgctggagacggtgcaggcgctgttgccggtgctgtgccaggcccacggcttgaccccccagcaggtggtggccatcgccagcaatggcggtggcaagcaggcgctggagacggtccagcggctgttgccggtgctgtgccaggcccacggcttgaccccggagcaggtggtggccatcgccagcaatattggtggcaagcaggcgctggagacggtgcaggcgctgttgccggtgctgtgccaggcccacggcttgaccccccagcaggtggtggccatcgccagcaatggcggtggcaagcaggcgctggagacggtccagcggctgttgccggtgctgtgccaggcccacggcttgaccccccagcaggtggtggccatcgccagcaataatggtggcaagcaggcgctggagacggtccagcggctgttgccggtgctgtgccaggcccacggcttgaccccggagcaggtggtggccatcgccagccacgatggcggcaagcaggcgctggagacggtccagcggctgttgccggtgctgtgccaggcccacggcttgaccccggagcaggtggtggccatcgccagcaatattggtggcaagcaggcgctggagacggtgcaggcgctgttgccggtgctgtgccaggcccacggcttgaccccccagcaggtggtggccatcgccagcaataatggtggcaagcaggcgctggagacggtccagcggctgttgccggtgctgtgccaggcccacggcttgaccccccagcaggtggtggccatcgccagcaataatggtggcaagcaggcgctggagacggtccagcggctgttgccggtgctgtgccaggcccacggcttgaccccggagcaggtggtggccatcgccagcaatattggtggcaagcaggcgctggagacggtgcaggcgctgttgccggtgctgtgccaggcccacggcttgaccccccagcaggtggtggccatcgccagcaatggcggtggcaagcaggcgctggagacggtccagcggctgttgccggtgctgtgccaggcccacggcttgaccccggagcaggtggtggccatcgccagcaatattggtggcaagcaggcgctggagacggtgcaggcgctgttgccggtgctgtgccaggcccacggcttgaccccccagcaggtggtggccatcgccagcaatggcggtggcaagcaggcgctggagacggtccagcggctgttgccggtgctgtgccaggcccacggcttgaccccccagcaggtggtggccatcgccagcaataatggtggcaagcaggcgctggagacggtccagcggctgttgccggtgctgtgccaggcccacggcttgacccctcagcaggtggtggccatcgccagcaatggcggcggcaggccggcgctggagagcattgttgcccagttatctcgccctgatccggcgttggccgcgttgaccaacgaccacctcgtcgccttggcctgcctcggcgggcgtcctgcgctggatgcagtgaaaaagggattgggggatcctatcagccgttcccagctggtgaagtccgagctggaggagaagaaatccgagttgaggcacaagctgaagtacgtgccccacgagtacatcgagctgatcgagatcgcccggaacagcacccaggaccgtatcctggagatgaaggtgatggagttcttcatgaaggtgtacggctacaggggcaagcacctgggcggctccaggaagcccgacggcgccatctacaccgtgggctcccccatcgactacggcgtgatcgtggacaccaaggcctactccggcggctacaacctgcccatcggccaggccgacgaaatgcagaggtacgtggaggagaaccagaccaggaacaagcacatcaaccccaacgagtggtggaaggtgtacccctccagcgtgaccgagttcaagttcctgttcgtgtccggccacttcaagggcaactacaaggcccagctgaccaggctgaaccacatcaccaactgcaacggcgccgtgctgtccgtggaggagctcctgatcggcggcgagatgatcaaggccggcaccctgaccctggaggaggtgaggaggaagttcaacaacggcgagatcaacttcgcggccgactgataa

SEQ ID NO: 30 - DNA, 2832 bp, Artificialsequence
  GRex5T3-R TALEN
atgggcgatcctaaaaagaaacgtaaggtcatcgataaggagaccgccgctgccaagttcgagagacagcacatggacagcatcgatatcgccgatctacgcacgctcggctacagccagcagcaacaggagaagatcaaaccgaaggttcgttcgacagtggcgcagcaccacgaggcactggtcggccacgggtttacacacgcgcacatcgttgcgttaagccaacacccggcagcgttagggaccgtcgctgtcaagtatcaggacatgatcgcagcgttgccagaggcgacacacgaagcgatcgttggcgtcggcaaacagtggtccggcgcacgcgctctggaggccttgctcacggtggcgggagagttgagaggtccaccgttacagttggacacaggccaacttctcaagattgcaaaacgtggcggcgtgaccgcagtggaggcagtgcatgcatggcgcaatgcactgacgggtgccccgctcaacttgaccccccagcaggtggtggccatcgccagcaataatggtggcaagcaggcgctggagacggtccagcggctgttgccggtgctgtgccaggcccacggcttgaccccggagcaggtggtggccatcgccagcaatattggtggcaagcaggcgctggagacggtgcaggcgctgttgccggtgctgtgccaggcccacggcttgaccccccagcaggtggtggccatcgccagcaatggcggtggcaagcaggcgctggagacggtccagcggctgttgccggtgctgtgccaggcccacggcttgaccccggagcaggtggtggccatcgccagccacgatggcggcaagcaggcgctggagacggtccagcggctgttgccggtgctgtgccaggcccacggcttgaccccggagcaggtggtggccatcgccagccacgatggcggcaagcaggcgctggagacggtccagcggctgttgccggtgctgtgccaggcccacggcttgaccccccagcaggtggtggccatcgccagcaatggcggtggcaagcaggcgctggagacggtccagcggctgttgccggtgctgtgccaggcccacggcttgaccccggagcaggtggtggccatcgccagccacgatggcggcaagcaggcgctggagacggtccagcggctgttgccggtgctgtgccaggcccacggcttgaccccggagcaggtggtggccatcgccagccacgatggcggcaagcaggcgctggagacggtccagcggctgttgccggtgctgtgccaggcccacggcttgaccccggagcaggtggtggccatcgccagcaatattggtggcaagcaggcgctggagacggtgcaggcgctgttgccggtgctgtgccaggcccacggcttgaccccggagcaggtggtggccatcgccagcaatattggtggcaagcaggcgctggagacggtgcaggcgctgttgccggtgctgtgccaggcccacggcttgaccccccagcaggtggtggccatcgccagcaataatggtggcaagcaggcgctggagacggtccagcggctgttgccggtgctgtgccaggcccacggcttgaccccccagcaggtggtggccatcgccagcaatggcggtggcaagcaggcgctggagacggtccagcggctgttgccggtgctgtgccaggcccacggcttgaccccccagcaggtggtggccatcgccagcaatggcggtggcaagcaggcgctggagacggtccagcggctgttgccggtgctgtgccaggcccacggcttgaccccccagcaggtggtggccatcgccagcaataatggtggcaagcaggcgctggagacggtccagcggctgttgccggtgctgtgccaggcccacggcttgaccccggagcaggtggtggccatcgccagcaatattggtggcaagcaggcgctggagacggtgcaggcgctgttgccggtgctgtgccaggcccacggcttgacccctcagcaggtggtggccatcgccagcaatggcggcggcaggccggcgctggagagcattgttgcccagttatctcgccctgatccggcgttggccgcgttgaccaacgaccacctcgtcgccttggcctgcctcggcgggcgtcctgcgctggatgcagtgaaaaagggattgggggatcctatcagccgttcccagctggtgaagtccgagctggaggagaagaaatccgagttgaggcacaagctgaagtacgtgccccacgagtacatcgagctgatcgagatcgcccggaacagcacccaggaccgtatcctggagatgaaggtgatggagttcttcatgaaggtgtacggctacaggggcaagcacctgggcggctccaggaagcccgacggcgccatctacaccgtgggctcccccatcgactacggcgtgatcgtggacaccaaggcctactccggcggctacaacctgcccatcggccaggccgacgaaatgcagaggtacgtggaggagaaccagaccaggaacaagcacatcaaccccaacgagtggtggaaggtgtacccctccagcgtgaccgagttcaagttcctgttcgtgtccggccacttcaagggcaactacaaggcccagctgaccaggctgaaccacatcaccaactgcaacggcgccgtgctgtccgtggaggagctcctgatcggcggcgagatgatcaaggccggcaccctgaccctggaggaggtgaggaggaagttcaacaacggcgagatcaacttcgcggccgactgataa

SEQ ID NO: 31 - DNA, 60 bp, Artificialsequence
  Forward primer GR exon 2
  misc_feature (31); (32); (33); (34); (35); (36); (37); (38); (39); (40): n is a or c or t or g
ccatctcatccctgcgtgtctccgactcagnnnnnnnnnnggttcatttaacaagctgcc

SEQ ID NO: 32 - DNA, 60 bp, Artificialsequence
  Forward primer GR exon 3
  misc_feature (31); (32); (33); (34); (35); (36); (37); (38); (39); (40): n is a or c or t or g
ccatctcatccctgcgtgtctccgactcagnnnnnnnnnngcattctgactatgaagtga

SEQ ID NO: 33 - DNA, 69 bp, Artificialsequence
  Forward primer GR exon 5
  misc_feature (31); (32); (33); (34); (35); (36); (37); (38); (39); (40): n is a or c or t or g
ccatctcatccctgcgtgtctccgactcagnnnnnnnnnntcagcaggccactacaggagtctcacaag

SEQ ID NO: 34 - DNA, 50 bp, Artificialsequence
  Reverse primer GR exon 2
cctatcccctgtgtgccttggcagtctcagagccagtgagggtgaagacg

SEQ ID NO: 35 - DNA, 50 bp, Artificialsequence
  Reverse primer GR exon 3
cctatcccctgtgtgccttggcagtctcaggggctttgcatataatggaa

SEQ ID NO: 36 - DNA, 59 bp, Artificialsequence
  Reverse primer GR exon 5
cctatcccctgtgtgccttggcagtctcagctgactctccccttcatagtccccagaac

SEQ ID NO: 37 - DNA, 49 bp, Artificialsequence
  TRAC_T01
ttgtcccacagatatccagaaccctgaccctgccgtgtaccagctgaga

SEQ ID NO: 38 - DNA, 49 bp, Artificialsequence
  TRBC_T01
tgtgtttgagccatcagaagcagagatctcccacacccaaaaggccaca

SEQ ID NO: 39 - DNA, 50 bp, Artificialsequence
  TRBC_T02
ttcccacccgaggtcgctgtgtttgagccatcagaagcagagatctccca

SEQ ID NO: 40 - DNA, 49 bp, Artificialsequence
  CD52_T02
ttcctcctactcaccatcagcctcctggttatggtacaggtaagagcaa

SEQ ID NO: 41 - protein, 530 aa, Artificialsequence
  Repeat TRAC_T01-L
LTPQQVVAIASNGGGKQALETVQRLLPVLCQAHGLTPQQVVAIASNNGGKQALETVQRLLPVLCQAHGLTPQQVVAIASNGGGKQALETVQRLLPVLCQAHGLTPEQVVAIASHDGGKQALETVQRLLPVLCQAHGLTPEQVVAIASHDGGKQALETVQRLLPVLCQAHGLTPEQVVAIASHDGGKQALETVQRLLPVLCQAHGLTPEQVVAIASNIGGKQALETVQALLPVLCQAHGLTPEQVVAIASHDGGKQALETVQRLLPVLCQAHGLTPEQVVAIASNIGGKQALETVQALLPVLCQAHGLTPQQVVAIASNNGGKQALETVQRLLPVLCQAHGLTPEQVVAIASNIGGKQALETVQALLPVLCQAHGLTPQQVVAIASNGGGKQALETVQRLLPVLCQAHGLTPEQVVAIASNIGGKQALETVQALLPVLCQAHGLTPQQVVAIASNGGGKQALETVQRLLPVLCQAHGLTPEQVVAIASHDGGKQALETVQRLLPVLCQAHGLTPQQVVAIASNGGGRPALE

SEQ ID NO: 42 - protein, 530 aa, Artificialsequence
  Repeat TRAC_T01-R
LTPEQVVAIASHDGGKQALETVQRLLPVLCQAHGLTPQQVVAIASNGGGKQALETVQRLLPVLCQAHGLTPEQVVAIASHDGGKQALETVQRLLPVLCQAHGLTPEQVVAIASNIGGKQALETVQALLPVLCQAHGLTPQQVVAIASNNGGKQALETVQRLLPVLCQAHGLTPEQVVAIASHDGGKQALETVQRLLPVLCQAHGLTPQQVVAIASNGGGKQALETVQRLLPVLCQAHGLTPQQVVAIASNNGGKQALETVQRLLPVLCQAHGLTPQQVVAIASNNGGKQALETVQRLLPVLCQAHGLTPQQVVAIASNGGGKQALETVQRLLPVLCQAHGLTPEQVVAIASNIGGKQALETVQALLPVLCQAHGLTPEQVVAIASHDGGKQALETVQRLLPVLCQAHGLTPEQVVAIASNIGGKQALETVQALLPVLCQAHGLTPEQVVAIASHDGGKQALETVQRLLPVLCQAHGLTPQQVVAIASNNGGKQALETVQRLLPVLCQAHGLTPQQVVAIASNGGGRPALE

SEQ ID NO: 43 - protein, 530 aa, Artificialsequence
  Repeat TRBC_T01-L
LTPQQVVAIASNNGGKQALETVQRLLPVLCQAHGLTPQQVVAIASNGGGKQALETVQRLLPVLCQAHGLTPQQVVAIASNNGGKQALETVQRLLPVLCQAHGLTPQQVVAIASNGGGKQALETVQRLLPVLCQAHGLTPQQVVAIASNGGGKQALETVQRLLPVLCQAHGLTPQQVVAIASNGGGKQALETVQRLLPVLCQAHGLTPQQVVAIASNNGGKQALETVQRLLPVLCQAHGLTPEQVVAIASNIGGKQALETVQALLPVLCQAHGLTPQQVVAIASNNGGKQALETVQRLLPVLCQAHGLTPEQVVAIASHDGGKQALETVQRLLPVLCQAHGLTPEQVVAIASHDGGKQALETVQRLLPVLCQAHGLTPEQVVAIASNIGGKQALETVQALLPVLCQAHGLTPQQVVAIASNGGGKQALETVQRLLPVLCQAHGLTPEQVVAIASHDGGKQALETVQRLLPVLCQAHGLTPEQVVAIASNIGGKQALETVQALLPVLCQAHGLTPQQVVAIASNGGGRPALE

SEQ ID NO: 44 - protein, 530 aa, Artificialsequence
  Repeat TRBC_T01-R
LTPQQVVAIASNNGGKQALETVQRLLPVLCQAHGLTPQQVVAIASNGGGKQALETVQRLLPVLCQAHGLTPQQVVAIASNNGGKQALETVQRLLPVLCQAHGLTPQQVVAIASNNGGKQALETVQRLLPVLCQAHGLTPEQVVAIASHDGGKQALETVQRLLPVLCQAHGLTPEQVVAIASHDGGKQALETVQRLLPVLCQAHGLTPQQVVAIASNGGGKQALETVQRLLPVLCQAHGLTPQQVVAIASNGGGKQALETVQRLLPVLCQAHGLTPQQVVAIASNGGGKQALETVQRLLPVLCQAHGLTPQQVVAIASNGGGKQALETVQRLLPVLCQAHGLTPQQVVAIASNNGGKQALETVQRLLPVLCQAHGLTPQQVVAIASNNGGKQALETVQRLLPVLCQAHGLTPQQVVAIASNNGGKQALETVQRLLPVLCQAHGLTPQQVVAIASNGGGKQALETVQRLLPVLCQAHGLTPQQVVAIASNNGGKQALETVQRLLPVLCQAHGLTPQQVVAIASNGGGRPALE

SEQ ID NO: 45 - protein, 530 aa, Artificialsequence
  Repeat TRBC_T02-L
LTPEQVVAIASHDGGKQALETVQRLLPVLCQAHGLTPEQVVAIASHDGGKQALETVQRLLPVLCQAHGLTPEQVVAIASHDGGKQALETVQRLLPVLCQAHGLTPEQVVAIASNIGGKQALETVQALLPVLCQAHGLTPEQVVAIASHDGGKQALETVQRLLPVLCQAHGLTPEQVVAIASHDGGKQALETVQRLLPVLCQAHGLTPEQVVAIASHDGGKQALETVQRLLPVLCQAHGLTPQQVVAIASNNGGKQALETVQRLLPVLCQAHGLTPEQVVAIASNIGGKQALETVQALLPVLCQAHGLTPQQVVAIASNNGGKQALETVQRLLPVLCQAHGLTPQQVVAIASNNGGKQALETVQRLLPVLCQAHGLTPQQVVAIASNGGGKQALETVQRLLPVLCQAHGLTPEQVVAIASHDGGKQALETVQRLLPVLCQAHGLTPQQVVAIASNNGGKQALETVQRLLPVLCQAHGLTPEQVVAIASHDGGKQALETVQRLLPVLCQAHGLTPQQVVAIASNGGGRPALE

SEQ ID NO: 46 - protein, 530 aa, Artificialsequence
  Repeat TRBC_T02-R
LTPQQVVAIASNNGGKQALETVQRLLPVLCQAHGLTPQQVVAIASNNGGKQALETVQRLLPVLCQAHGLTPQQVVAIASNNGGKQALETVQRLLPVLCQAHGLTPEQVVAIASNIGGKQALETVQALLPVLCQAHGLTPQQVVAIASNNGGKQALETVQRLLPVLCQAHGLTPEQVVAIASNIGGKQALETVQALLPVLCQAHGLTPQQVVAIASNGGGKQALETVQRLLPVLCQAHGLTPEQVVAIASHDGGKQALETVQRLLPVLCQAHGLTPQQVVAIASNGGGKQALETVQRLLPVLCQAHGLTPEQVVAIASHDGGKQALETVQRLLPVLCQAHGLTPQQVVAIASNGGGKQALETVQRLLPVLCQAHGLTPQQVVAIASNNGGKQALETVQRLLPVLCQAHGLTPEQVVAIASHDGGKQALETVQRLLPVLCQAHGLTPQQVVAIASNGGGKQALETVQRLLPVLCQAHGLTPQQVVAIASNGGGKQALETVQRLLPVLCQAHGLTPQQVVAIASNGGGRPALE

SEQ ID NO: 47 - protein, 530 aa, Artificialsequence
  Repeat CD52_T02-L
LTPQQVVAIASNGGGKQALETVQRLLPVLCQAHGLTPEQVVAIASHDGGKQALETVQRLLPVLCQAHGLTPEQVVAIASHDGGKQALETVQRLLPVLCQAHGLTPQQVVAIASNGGGKQALETVQRLLPVLCQAHGLTPEQVVAIASHDGGKQALETVQRLLPVLCQAHGLTPEQVVAIASHDGGKQALETVQRLLPVLCQAHGLTPQQVVAIASNGGGKQALETVQRLLPVLCQAHGLTPEQVVAIASNIGGKQALETVQALLPVLCQAHGLTPEQVVAIASHDGGKQALETVQRLLPVLCQAHGLTPQQVVAIASNGGGKQALETVQRLLPVLCQAHGLTPEQVVAIASHDGGKQALETVQRLLPVLCQAHGLTPEQVVAIASNIGGKQALETVQALLPVLCQAHGLTPEQVVAIASHDGGKQALETVQRLLPVLCQAHGLTPEQVVAIASHDGGKQALETVQRLLPVLCQAHGLTPEQVVAIASNIGGKQALETVQALLPVLCQAHGLTPQQVVAIASNGGGRPALE

SEQ ID NO: 48 - protein, 530 aa, Artificialsequence
  Repeat CD52_T02-R
LTPQQVVAIASNGGGKQALETVQRLLPVLCQAHGLTPQQVVAIASNNGGKQALETVQRLLPVLCQAHGLTPEQVVAIASHDGGKQALETVQRLLPVLCQAHGLTPQQVVAIASNGGGKQALETVQRLLPVLCQAHGLTPEQVVAIASHDGGKQALETVQRLLPVLCQAHGLTPQQVVAIASNGGGKQALETVQRLLPVLCQAHGLTPQQVVAIASNGGGKQALETVQRLLPVLCQAHGLTPEQVVAIASNIGGKQALETVQALLPVLCQAHGLTPEQVVAIASHDGGKQALETVQRLLPVLCQAHGLTPEQVVAIASHDGGKQALETVQRLLPVLCQAHGLTPQQVVAIASNGGGKQALETVQRLLPVLCQAHGLTPQQVVAIASNNGGKQALETVQRLLPVLCQAHGLTPQQVVAIASNGGGKQALETVQRLLPVLCQAHGLTPEQVVAIASNIGGKQALETVQALLPVLCQAHGLTPEQVVAIASHDGGKQALETVQRLLPVLCQAHGLTPQQVVAIASNGGGRPALE

SEQ ID NO: 49 - DNA, 2814 bp, Artificialsequence
  TRAC_T01-L TALEN
atgggcgatcctaaaaagaaacgtaaggtcatcgattacccatacgatgttccagattacgctatcgatatcgccgatctacgcacgctcggctacagccagcagcaacaggagaagatcaaaccgaaggttcgttcgacagtggcgcagcaccacgaggcactggtcggccacgggtttacacacgcgcacatcgttgcgttaagccaacacccggcagcgttagggaccgtcgctgtcaagtatcaggacatgatcgcagcgttgccagaggcgacacacgaagcgatcgttggcgtcggcaaacagtggtccggcgcacgcgctctggaggccttgctcacggtggcgggagagttgagaggtccaccgttacagttggacacaggccaacttctcaagattgcaaaacgtggcggcgtgaccgcagtggaggcagtgcatgcatggcgcaatgcactgacgggtgccccgctcaacttgaccccccagcaggtggtggccatcgccagcaatggcggtggcaagcaggcgctggagacggtccagcggctgttgccggtgctgtgccaggcccacggcttgaccccccagcaggtggtggccatcgccagcaataatggtggcaagcaggcgctggagacggtccagcggctgttgccggtgctgtgccaggcccacggcttgaccccccagcaggtggtggccatcgccagcaatggcggtggcaagcaggcgctggagacggtccagcggctgttgccggtgctgtgccaggcccacggcttgaccccggagcaggtggtggccatcgccagccacgatggcggcaagcaggcgctggagacggtccagcggctgttgccggtgctgtgccaggcccacggcttgaccccggagcaggtggtggccatcgccagccacgatggcggcaagcaggcgctggagacggtccagcggctgttgccggtgctgtgccaggcccacggcttgaccccggagcaggtggtggccatcgccagccacgatggcggcaagcaggcgctggagacggtccagcggctgttgccggtgctgtgccaggcccacggcttgaccccggagcaggtggtggccatcgccagcaatattggtggcaagcaggcgctggagacggtgcaggcgctgttgccggtgctgtgccaggcccacggcttgaccccggagcaggtggtggccatcgccagccacgatggcggcaagcaggcgctggagacggtccagcggctgttgccggtgctgtgccaggcccacggcttgaccccggagcaggtggtggccatcgccagcaatattggtggcaagcaggcgctggagacggtgcaggcgctgttgccggtgctgtgccaggcccacggcttgaccccccagcaggtggtggccatcgccagcaataatggtggcaagcaggcgctggagacggtccagcggctgttgccggtgctgtgccaggcccacggcttgaccccggagcaggtggtggccatcgccagcaatattggtggcaagcaggcgctggagacggtgcaggcgctgttgccggtgctgtgccaggcccacggcttgaccccccagcaggtggtggccatcgccagcaatggcggtggcaagcaggcgctggagacggtccagcggctgttgccggtgctgtgccaggcccacggcttgaccccggagcaggtggtggccatcgccagcaatattggtggcaagcaggcgctggagacggtgcaggcgctgttgccggtgctgtgccaggcccacggcttgaccccccagcaggtggtggccatcgccagcaatggcggtggcaagcaggcgctggagacggtccagcggctgttgccggtgctgtgccaggcccacggcttgaccccggagcaggtggtggccatcgccagccacgatggcggcaagcaggcgctggagacggtccagcggctgttgccggtgctgtgccaggcccacggcttgacccctcagcaggtggtggccatcgccagcaatggcggcggcaggccggcgctggagagcattgttgcccagttatctcgccctgatccggcgttggccgcgttgaccaacgaccacctcgtcgccttggcctgcctcggcgggcgtcctgcgctggatgcagtgaaaaagggattgggggatcctatcagccgttcccagctggtgaagtccgagctggaggagaagaaatccgagttgaggcacaagctgaagtacgtgccccacgagtacatcgagctgatcgagatcgcccggaacagcacccaggaccgtatcctggagatgaaggtgatggagttcttcatgaaggtgtacggctacaggggcaagcacctgggcggctccaggaagcccgacggcgccatctacaccgtgggctcccccatcgactacggcgtgatcgtggacaccaaggcctactccggcggctacaacctgcccatcggccaggccgacgaaatgcagaggtacgtggaggagaaccagaccaggaacaagcacatcaaccccaacgagtggtggaaggtgtacccctccagcgtgaccgagttcaagttcctgttcgtgtccggccacttcaagggcaactacaaggcccagctgaccaggctgaaccacatcaccaactgcaacggcgccgtgctgtccgtggaggagctcctgatcggcggcgagatgatcaaggccggcaccctgaccctggaggaggtgaggaggaagttcaacaacggcgagatcaacttcgcggccgactgataa

SEQ ID NO: 50 - DNA, 2832 bp, Artificialsequence
  TRAC_T01-R TALEN
atgggcgatcctaaaaagaaacgtaaggtcatcgataaggagaccgccgctgccaagttcgagagacagcacatggacagcatcgatatcgccgatctacgcacgctcggctacagccagcagcaacaggagaagatcaaaccgaaggttcgttcgacagtggcgcagcaccacgaggcactggtcggccacgggtttacacacgcgcacatcgttgcgttaagccaacacccggcagcgttagggaccgtcgctgtcaagtatcaggacatgatcgcagcgttgccagaggcgacacacgaagcgatcgttggcgtcggcaaacagtggtccggcgcacgcgctctggaggccttgctcacggtggcgggagagttgagaggtccaccgttacagttggacacaggccaacttctcaagattgcaaaacgtggcggcgtgaccgcagtggaggcagtgcatgcatggcgcaatgcactgacgggtgccccgctcaacttgaccccggagcaggtggtggccatcgccagccacgatggcggcaagcaggcgctggagacggtccagcggctgttgccggtgctgtgccaggcccacggcttgaccccccagcaggtggtggccatcgccagcaatggcggtggcaagcaggcgctggagacggtccagcggctgttgccggtgctgtgccaggcccacggcttgaccccggagcaggtggtggccatcgccagccacgatggcggcaagcaggcgctggagacggtccagcggctgttgccggtgctgtgccaggcccacggcttgaccccggagcaggtggtggccatcgccagcaatattggtggcaagcaggcgctggagacggtgcaggcgctgttgccggtgctgtgccaggcccacggcttgaccccccagcaggtggtggccatcgccagcaataatggtggcaagcaggcgctggagacggtccagcggctgttgccggtgctgtgccaggcccacggcttgaccccggagcaggtggtggccatcgccagccacgatggcggcaagcaggcgctggagacggtccagcggctgttgccggtgctgtgccaggcccacggcttgaccccccagcaggtggtggccatcgccagcaatggcggtggcaagcaggcgctggagacggtccagcggctgttgccggtgctgtgccaggcccacggcttgaccccccagcaggtggtggccatcgccagcaataatggtggcaagcaggcgctggagacggtccagcggctgttgccggtgctgtgccaggcccacggcttgaccccccagcaggtggtggccatcgccagcaataatggtggcaagcaggcgctggagacggtccagcggctgttgccggtgctgtgccaggcccacggcttgaccccccagcaggtggtggccatcgccagcaatggcggtggcaagcaggcgctggagacggtccagcggctgttgccggtgctgtgccaggcccacggcttgaccccggagcaggtggtggccatcgccagcaatattggtggcaagcaggcgctggagacggtgcaggcgctgttgccggtgctgtgccaggcccacggcttgaccccggagcaggtggtggccatcgccagccacgatggcggcaagcaggcgctggagacggtccagcggctgttgccggtgctgtgccaggcccacggcttgaccccggagcaggtggtggccatcgccagcaatattggtggcaagcaggcgctggagacggtgcaggcgctgttgccggtgctgtgccaggcccacggcttgaccccggagcaggtggtggccatcgccagccacgatggcggcaagcaggcgctggagacggtccagcggctgttgccggtgctgtgccaggcccacggcttgaccccccagcaggtggtggccatcgccagcaataatggtggcaagcaggcgctggagacggtccagcggctgttgccggtgctgtgccaggcccacggcttgacccctcagcaggtggtggccatcgccagcaatggcggcggcaggccggcgctggagagcattgttgcccagttatctcgccctgatccggcgttggccgcgttgaccaacgaccacctcgtcgccttggcctgcctcggcgggcgtcctgcgctggatgcagtgaaaaagggattgggggatcctatcagccgttcccagctggtgaagtccgagctggaggagaagaaatccgagttgaggcacaagctgaagtacgtgccccacgagtacatcgagctgatcgagatcgcccggaacagcacccaggaccgtatcctggagatgaaggtgatggagttcttcatgaaggtgtacggctacaggggcaagcacctgggcggctccaggaagcccgacggcgccatctacaccgtgggctcccccatcgactacggcgtgatcgtggacaccaaggcctactccggcggctacaacctgcccatcggccaggccgacgaaatgcagaggtacgtggaggagaaccagaccaggaacaagcacatcaaccccaacgagtggtggaaggtgtacccctccagcgtgaccgagttcaagttcctgttcgtgtccggccacttcaagggcaactacaaggcccagctgaccaggctgaaccacatcaccaactgcaacggcgccgtgctgtccgtggaggagctcctgatcggcggcgagatgatcaaggccggcaccctgaccctggaggaggtgaggaggaagttcaacaacggcgagatcaacttcgcggccgactgataa

SEQ ID NO: 51 - DNA, 2814 bp, Artificialsequence
  TRBC_T01-L TALEN
atgggcgatcctaaaaagaaacgtaaggtcatcgattacccatacgatgttccagattacgctatcgatatcgccgatctacgcacgctcggctacagccagcagcaacaggagaagatcaaaccgaaggttcgttcgacagtggcgcagcaccacgaggcactggtcggccacgggtttacacacgcgcacatcgttgcgttaagccaacacccggcagcgttagggaccgtcgctgtcaagtatcaggacatgatcgcagcgttgccagaggcgacacacgaagcgatcgttggcgtcggcaaacagtggtccggcgcacgcgctctggaggccttgctcacggtggcgggagagttgagaggtccaccgttacagttggacacaggccaacttctcaagattgcaaaacgtggcggcgtgaccgcagtggaggcagtgcatgcatggcgcaatgcactgacgggtgccccgctcaacttgaccccccagcaggtggtggccatcgccagcaataatggtggcaagcaggcgctggagacggtccagcggctgttgccggtgctgtgccaggcccacggcttgaccccccagcaggtggtggccatcgccagcaatggcggtggcaagcaggcgctggagacggtccagcggctgttgccggtgctgtgccaggcccacggcttgaccccccagcaggtggtggccatcgccagcaataatggtggcaagcaggcgctggagacggtccagcggctgttgccggtgctgtgccaggcccacggcttgaccccccagcaggtggtggccatcgccagcaatggcggtggcaagcaggcgctggagacggtccagcggctgttgccggtgctgtgccaggcccacggcttgaccccccagcaggtggtggccatcgccagcaatggcggtggcaagcaggcgctggagacggtccagcggctgttgccggtgctgtgccaggcccacggcttgaccccccagcaggtggtggccatcgccagcaatggcggtggcaagcaggcgctggagacggtccagcggctgttgccggtgctgtgccaggcccacggcttgaccccccagcaggtggtggccatcgccagcaataatggtggcaagcaggcgctggagacggtccagcggctgttgccggtgctgtgccaggcccacggcttgaccccggagcaggtggtggccatcgccagcaatattggtggcaagcaggcgctggagacggtgcaggcgctgttgccggtgctgtgccaggcccacggcttgaccccccagcaggtggtggccatcgccagcaataatggtggcaagcaggcgctggagacggtccagcggctgttgccggtgctgtgccaggcccacggcttgaccccggagcaggtggtggccatcgccagccacgatggcggcaagcaggcgctggagacggtccagcggctgttgccggtgctgtgccaggcccacggcttgaccccggagcaggtggtggccatcgccagccacgatggcggcaagcaggcgctggagacggtccagcggctgttgccggtgctgtgccaggcccacggcttgaccccggagcaggtggtggccatcgccagcaatattggtggcaagcaggcgctggagacggtgcaggcgctgttgccggtgctgtgccaggcccacggcttgaccccccagcaggtggtggccatcgccagcaatggcggtggcaagcaggcgctggagacggtccagcggctgttgccggtgctgtgccaggcccacggcttgaccccggagcaggtggtggccatcgccagccacgatggcggcaagcaggcgctggagacggtccagcggctgttgccggtgctgtgccaggcccacggcttgaccccggagcaggtggtggccatcgccagcaatattggtggcaagcaggcgctggagacggtgcaggcgctgttgccggtgctgtgccaggcccacggcttgacccctcagcaggtggtggccatcgccagcaatggcggcggcaggccggcgctggagagcattgttgcccagttatctcgccctgatccggcgttggccgcgttgaccaacgaccacctcgtcgccttggcctgcctcggcgggcgtcctgcgctggatgcagtgaaaaagggattgggggatcctatcagccgttcccagctggtgaagtccgagctggaggagaagaaatccgagttgaggcacaagctgaagtacgtgccccacgagtacatcgagctgatcgagatcgcccggaacagcacccaggaccgtatcctggagatgaaggtgatggagttcttcatgaaggtgtacggctacaggggcaagcacctgggcggctccaggaagcccgacggcgccatctacaccgtgggctcccccatcgactacggcgtgatcgtggacaccaaggcctactccggcggctacaacctgcccatcggccaggccgacgaaatgcagaggtacgtggaggagaaccagaccaggaacaagcacatcaaccccaacgagtggtggaaggtgtacccctccagcgtgaccgagttcaagttcctgttcgtgtccggccacttcaagggcaactacaaggcccagctgaccaggctgaaccacatcaccaactgcaacggcgccgtgctgtccgtggaggagctcctgatcggcggcgagatgatcaaggccggcaccctgaccctggaggaggtgaggaggaagttcaacaacggcgagatcaacttcgcggccgactgataa

SEQ ID NO: 52 - DNA, 2832 bp, Artificialsequence
  TRBC_T01-R TALEN
atgggcgatcctaaaaagaaacgtaaggtcatcgataaggagaccgccgctgccaagttcgagagacagcacatggacagcatcgatatcgccgatctacgcacgctcggctacagccagcagcaacaggagaagatcaaaccgaaggttcgttcgacagtggcgcagcaccacgaggcactggtcggccacgggtttacacacgcgcacatcgttgcgttaagccaacacccggcagcgttagggaccgtcgctgtcaagtatcaggacatgatcgcagcgttgccagaggcgacacacgaagcgatcgttggcgtcggcaaacagtggtccggcgcacgcgctctggaggccttgctcacggtggcgggagagttgagaggtccaccgttacagttggacacaggccaacttctcaagattgcaaaacgtggcggcgtgaccgcagtggaggcagtgcatgcatggcgcaatgcactgacgggtgccccgctcaacttgaccccccagcaggtggtggccatcgccagcaataatggtggcaagcaggcgctggagacggtccagcggctgttgccggtgctgtgccaggcccacggcttgaccccccagcaggtggtggccatcgccagcaatggcggtggcaagcaggcgctggagacggtccagcggctgttgccggtgctgtgccaggcccacggcttgaccccccagcaggtggtggccatcgccagcaataatggtggcaagcaggcgctggagacggtccagcggctgttgccggtgctgtgccaggcccacggcttgaccccccagcaggtggtggccatcgccagcaataatggtggcaagcaggcgctggagacggtccagcggctgttgccggtgctgtgccaggcccacggcttgaccccggagcaggtggtggccatcgccagccacgatggcggcaagcaggcgctggagacggtccagcggctgttgccggtgctgtgccaggcccacggcttgaccccggagcaggtggtggccatcgccagccacgatggcggcaagcaggcgctggagacggtccagcggctgttgccggtgctgtgccaggcccacggcttgaccccccagcaggtggtggccatcgccagcaatggcggtggcaagcaggcgctggagacggtccagcggctgttgccggtgctgtgccaggcccacggcttgaccccccagcaggtggtggccatcgccagcaatggcggtggcaagcaggcgctggagacggtccagcggctgttgccggtgctgtgccaggcccacggcttgaccccccagcaggtggtggccatcgccagcaatggcggtggcaagcaggcgctggagacggtccagcggctgttgccggtgctgtgccaggcccacggcttgaccccccagcaggtggtggccatcgccagcaatggcggtggcaagcaggcgctggagacggtccagcggctgttgccggtgctgtgccaggcccacggcttgaccccccagcaggtggtggccatcgccagcaataatggtggcaagcaggcgctggagacggtccagcggctgttgccggtgctgtgccaggcccacggcttgaccccccagcaggtggtggccatcgccagcaataatggtggcaagcaggcgctggagacggtccagcggctgttgccggtgctgtgccaggcccacggcttgaccccccagcaggtggtggccatcgccagcaataatggtggcaagcaggcgctggagacggtccagcggctgttgccggtgctgtgccaggcccacggcttgaccccccagcaggtggtggccatcgccagcaatggcggtggcaagcaggcgctggagacggtccagcggctgttgccggtgctgtgccaggcccacggcttgaccccccagcaggtggtggccatcgccagcaataatggtggcaagcaggcgctggagacggtccagcggctgttgccggtgctgtgccaggcccacggcttgacccctcagcaggtggtggccatcgccagcaatggcggcggcaggccggcgctggagagcattgttgcccagttatctcgccctgatccggcgttggccgcgttgaccaacgaccacctcgtcgccttggcctgcctcggcgggcgtcctgcgctggatgcagtgaaaaagggattgggggatcctatcagccgttcccagctggtgaagtccgagctggaggagaagaaatccgagttgaggcacaagctgaagtacgtgccccacgagtacatcgagctgatcgagatcgcccggaacagcacccaggaccgtatcctggagatgaaggtgatggagttcttcatgaaggtgtacggctacaggggcaagcacctgggcggctccaggaagcccgacggcgccatctacaccgtgggctcccccatcgactacggcgtgatcgtggacaccaaggcctactccggcggctacaacctgcccatcggccaggccgacgaaatgcagaggtacgtggaggagaaccagaccaggaacaagcacatcaaccccaacgagtggtggaaggtgtacccctccagcgtgaccgagttcaagttcctgttcgtgtccggccacttcaagggcaactacaaggcccagctgaccaggctgaaccacatcaccaactgcaacggcgccgtgctgtccgtggaggagctcctgatcggcggcgagatgatcaaggccggcaccctgaccctggaggaggtgaggaggaagttcaacaacggcgagatcaacttcgcggccgactgataa

SEQ ID NO: 53 - DNA, 2814 bp, Artificialsequence
  TRBC_T02-L TALEN
atgggcgatcctaaaaagaaacgtaaggtcatcgattacccatacgatgttccagattacgctatcgatatcgccgatctacgcacgctcggctacagccagcagcaacaggagaagatcaaaccgaaggttcgttcgacagtggcgcagcaccacgaggcactggtcggccacgggtttacacacgcgcacatcgttgcgttaagccaacacccggcagcgttagggaccgtcgctgtcaagtatcaggacatgatcgcagcgttgccagaggcgacacacgaagcgatcgttggcgtcggcaaacagtggtccggcgcacgcgctctggaggccttgctcacggtggcgggagagttgagaggtccaccgttacagttggacacaggccaacttctcaagattgcaaaacgtggcggcgtgaccgcagtggaggcagtgcatgcatggcgcaatgcactgacgggtgccccgctcaacttgaccccggagcaggtggtggccatcgccagccacgatggcggcaagcaggcgctggagacggtccagcggctgttgccggtgctgtgccaggcccacggcttgaccccggagcaggtggtggccatcgccagccacgatggcggcaagcaggcgctggagacggtccagcggctgttgccggtgctgtgccaggcccacggcttgaccccggagcaggtggtggccatcgccagccacgatggcggcaagcaggcgctggagacggtccagcggctgttgccggtgctgtgccaggcccacggcttgaccccggagcaggtggtggccatcgccagcaatattggtggcaagcaggcgctggagacggtgcaggcgctgttgccggtgctgtgccaggcccacggcttgaccccggagcaggtggtggccatcgccagccacgatggcggcaagcaggcgctggagacggtccagcggctgttgccggtgctgtgccaggcccacggcttgaccccggagcaggtggtggccatcgccagccacgatggcggcaagcaggcgctggagacggtccagcggctgttgccggtgctgtgccaggcccacggcttgaccccggagcaggtggtggccatcgccagccacgatggcggcaagcaggcgctggagacggtccagcggctgttgccggtgctgtgccaggcccacggcttgaccccccagcaggtggtggccatcgccagcaataatggtggcaagcaggcgctggagacggtccagcggctgttgccggtgctgtgccaggcccacggcttgaccccggagcaggtggtggccatcgccagcaatattggtggcaagcaggcgctggagacggtgcaggcgctgttgccggtgctgtgccaggcccacggcttgaccccccagcaggtggtggccatcgccagcaataatggtggcaagcaggcgctggagacggtccagcggctgttgccggtgctgtgccaggcccacggcttgaccccccagcaggtggtggccatcgccagcaataatggtggcaagcaggcgctggagacggtccagcggctgttgccggtgctgtgccaggcccacggcttgaccccccagcaggtggtggccatcgccagcaatggcggtggcaagcaggcgctggagacggtccagcggctgttgccggtgctgtgccaggcccacggcttgaccccggagcaggtggtggccatcgccagccacgatggcggcaagcaggcgctggagacggtccagcggctgttgccggtgctgtgccaggcccacggcttgaccccccagcaggtggtggccatcgccagcaataatggtggcaagcaggcgctggagacggtccagcggctgttgccggtgctgtgccaggcccacggcttgaccccggagcaggtggtggccatcgccagccacgatggcggcaagcaggcgctggagacggtccagcggctgttgccggtgctgtgccaggcccacggcttgacccctcagcaggtggtggccatcgccagcaatggcggcggcaggccggcgctggagagcattgttgcccagttatctcgccctgatccggcgttggccgcgttgaccaacgaccacctcgtcgccttggcctgcctcggcgggcgtcctgcgctggatgcagtgaaaaagggattgggggatcctatcagccgttcccagctggtgaagtccgagctggaggagaagaaatccgagttgaggcacaagctgaagtacgtgccccacgagtacatcgagctgatcgagatcgcccggaacagcacccaggaccgtatcctggagatgaaggtgatggagttcttcatgaaggtgtacggctacaggggcaagcacctgggcggctccaggaagcccgacggcgccatctacaccgtgggctcccccatcgactacggcgtgatcgtggacaccaaggcctactccggcggctacaacctgcccatcggccaggccgacgaaatgcagaggtacgtggaggagaaccagaccaggaacaagcacatcaaccccaacgagtggtggaaggtgtacccctccagcgtgaccgagttcaagttcctgttcgtgtccggccacttcaagggcaactacaaggcccagctgaccaggctgaaccacatcaccaactgcaacggcgccgtgctgtccgtggaggagctcctgatcggcggcgagatgatcaaggccggcaccctgaccctggaggaggtgaggaggaagttcaacaacggcgagatcaacttcgcggccgactgataa

SEQ ID NO: 54 - DNA, 2832 bp, Artificialsequence
  TRBC_T02-R TALEN
atgggcgatcctaaaaagaaacgtaaggtcatcgataaggagaccgccgctgccaagttcgagagacagcacatggacagcatcgatatcgccgatctacgcacgctcggctacagccagcagcaacaggagaagatcaaaccgaaggttcgttcgacagtggcgcagcaccacgaggcactggtcggccacgggtttacacacgcgcacatcgttgcgttaagccaacacccggcagcgttagggaccgtcgctgtcaagtatcaggacatgatcgcagcgttgccagaggcgacacacgaagcgatcgttggcgtcggcaaacagtggtccggcgcacgcgctctggaggccttgctcacggtggcgggagagttgagaggtccaccgttacagttggacacaggccaacttctcaagattgcaaaacgtggcggcgtgaccgcagtggaggcagtgcatgcatggcgcaatgcactgacgggtgccccgctcaacttgaccccccagcaggtggtggccatcgccagcaataatggtggcaagcaggcgctggagacggtccagcggctgttgccggtgctgtgccaggcccacggcttgaccccccagcaggtggtggccatcgccagcaataatggtggcaagcaggcgctggagacggtccagcggctgttgccggtgctgtgccaggcccacggcttgaccccccagcaggtggtggccatcgccagcaataatggtggcaagcaggcgctggagacggtccagcggctgttgccggtgctgtgccaggcccacggcttgaccccggagcaggtggtggccatcgccagcaatattggtggcaagcaggcgctggagacggtgcaggcgctgttgccggtgctgtgccaggcccacggcttgaccccccagcaggtggtggccatcgccagcaataatggtggcaagcaggcgctggagacggtccagcggctgttgccggtgctgtgccaggcccacggcttgaccccggagcaggtggtggccatcgccagcaatattggtggcaagcaggcgctggagacggtgcaggcgctgttgccggtgctgtgccaggcccacggcttgaccccccagcaggtggtggccatcgccagcaatggcggtggcaagcaggcgctggagacggtccagcggctgttgccggtgctgtgccaggcccacggcttgaccccggagcaggtggtggccatcgccagccacgatggcggcaagcaggcgctggagacggtccagcggctgttgccggtgctgtgccaggcccacggcttgaccccccagcaggtggtggccatcgccagcaatggcggtggcaagcaggcgctggagacggtccagcggctgttgccggtgctgtgccaggcccacggcttgaccccggagcaggtggtggccatcgccagccacgatggcggcaagcaggcgctggagacggtccagcggctgttgccggtgctgtgccaggcccacggcttgaccccccagcaggtggtggccatcgccagcaatggcggtggcaagcaggcgctggagacggtccagcggctgttgccggtgctgtgccaggcccacggcttgaccccccagcaggtggtggccatcgccagcaataatggtggcaagcaggcgctggagacggtccagcggctgttgccggtgctgtgccaggcccacggcttgaccccggagcaggtggtggccatcgccagccacgatggcggcaagcaggcgctggagacggtccagcggctgttgccggtgctgtgccaggcccacggcttgaccccccagcaggtggtggccatcgccagcaatggcggtggcaagcaggcgctggagacggtccagcggctgttgccggtgctgtgccaggcccacggcttgaccccccagcaggtggtggccatcgccagcaatggcggtggcaagcaggcgctggagacggtccagcggctgttgccggtgctgtgccaggcccacggcttgacccctcagcaggtggtggccatcgccagcaatggcggcggcaggccggcgctggagagcattgttgcccagttatctcgccctgatccggcgttggccgcgttgaccaacgaccacctcgtcgccttggcctgcctcggcgggcgtcctgcgctggatgcagtgaaaaagggattgggggatcctatcagccgttcccagctggtgaagtccgagctggaggagaagaaatccgagttgaggcacaagctgaagtacgtgccccacgagtacatcgagctgatcgagatcgcccggaacagcacccaggaccgtatcctggagatgaaggtgatggagttcttcatgaaggtgtacggctacaggggcaagcacctgggcggctccaggaagcccgacggcgccatctacaccgtgggctcccccatcgactacggcgtgatcgtggacaccaaggcctactccggcggctacaacctgcccatcggccaggccgacgaaatgcagaggtacgtggaggagaaccagaccaggaacaagcacatcaaccccaacgagtggtggaaggtgtacccctccagcgtgaccgagttcaagttcctgttcgtgtccggccacttcaagggcaactacaaggcccagctgaccaggctgaaccacatcaccaactgcaacggcgccgtgctgtccgtggaggagctcctgatcggcggcgagatgatcaaggccggcaccctgaccctggaggaggtgaggaggaagttcaacaacggcgagatcaacttcgcggccgactgataa

SEQ ID NO: 55 - DNA, 2814 bp, Artificialsequence
  CD52_T02-L TALEN
atgggcgatcctaaaaagaaacgtaaggtcatcgattacccatacgatgttccagattacgctatcgatatcgccgatctacgcacgctcggctacagccagcagcaacaggagaagatcaaaccgaaggttcgttcgacagtggcgcagcaccacgaggcactggtcggccacgggtttacacacgcgcacatcgttgcgttaagccaacacccggcagcgttagggaccgtcgctgtcaagtatcaggacatgatcgcagcgttgccagaggcgacacacgaagcgatcgttggcgtcggcaaacagtggtccggcgcacgcgctctggaggccttgctcacggtggcgggagagttgagaggtccaccgttacagttggacacaggccaacttctcaagattgcaaaacgtggcggcgtgaccgcagtggaggcagtgcatgcatggcgcaatgcactgacgggtgccccgctcaacttgaccccccagcaggtggtggccatcgccagcaatggcggtggcaagcaggcgctggagacggtccagcggctgttgccggtgctgtgccaggcccacggcttgaccccggagcaggtggtggccatcgccagccacgatggcggcaagcaggcgctggagacggtccagcggctgttgccggtgctgtgccaggcccacggcttgaccccggagcaggtggtggccatcgccagccacgatggcggcaagcaggcgctggagacggtccagcggctgttgccggtgctgtgccaggcccacggcttgaccccccagcaggtggtggccatcgccagcaatggcggtggcaagcaggcgctggagacggtccagcggctgttgccggtgctgtgccaggcccacggcttgaccccggagcaggtggtggccatcgccagccacgatggcggcaagcaggcgctggagacggtccagcggctgttgccggtgctgtgccaggcccacggcttgaccccggagcaggtggtggccatcgccagccacgatggcggcaagcaggcgctggagacggtccagcggctgttgccggtgctgtgccaggcccacggcttgaccccccagcaggtggtggccatcgccagcaatggcggtggcaagcaggcgctggagacggtccagcggctgttgccggtgctgtgccaggcccacggcttgaccccggagcaggtggtggccatcgccagcaatattggtggcaagcaggcgctggagacggtgcaggcgctgttgccggtgctgtgccaggcccacggcttgaccccggagcaggtggtggccatcgccagccacgatggcggcaagcaggcgctggagacggtccagcggctgttgccggtgctgtgccaggcccacggcttgaccccccagcaggtggtggccatcgccagcaatggcggtggcaagcaggcgctggagacggtccagcggctgttgccggtgctgtgccaggcccacggcttgaccccggagcaggtggtggccatcgccagccacgatggcggcaagcaggcgctggagacggtccagcggctgttgccggtgctgtgccaggcccacggcttgaccccggagcaggtggtggccatcgccagcaatattggtggcaagcaggcgctggagacggtgcaggcgctgttgccggtgctgtgccaggcccacggcttgaccccggagcaggtggtggccatcgccagccacgatggcggcaagcaggcgctggagacggtccagcggctgttgccggtgctgtgccaggcccacggcttgaccccggagcaggtggtggccatcgccagccacgatggcggcaagcaggcgctggagacggtccagcggctgttgccggtgctgtgccaggcccacggcttgaccccggagcaggtggtggccatcgccagcaatattggtggcaagcaggcgctggagacggtgcaggcgctgttgccggtgctgtgccaggcccacggcttgacccctcagcaggtggtggccatcgccagcaatggcggcggcaggccggcgctggagagcattgttgcccagttatctcgccctgatccggcgttggccgcgttgaccaacgaccacctcgtcgccttggcctgcctcggcgggcgtcctgcgctggatgcagtgaaaaagggattgggggatcctatcagccgttcccagctggtgaagtccgagctggaggagaagaaatccgagttgaggcacaagctgaagtacgtgccccacgagtacatcgagctgatcgagatcgcccggaacagcacccaggaccgtatcctggagatgaaggtgatggagttcttcatgaaggtgtacggctacaggggcaagcacctgggcggctccaggaagcccgacggcgccatctacaccgtgggctcccccatcgactacggcgtgatcgtggacaccaaggcctactccggcggctacaacctgcccatcggccaggccgacgaaatgcagaggtacgtggaggagaaccagaccaggaacaagcacatcaaccccaacgagtggtggaaggtgtacccctccagcgtgaccgagttcaagttcctgttcgtgtccggccacttcaagggcaactacaaggcccagctgaccaggctgaaccacatcaccaactgcaacggcgccgtgctgtccgtggaggagctcctgatcggcggcgagatgatcaaggccggcaccctgaccctggaggaggtgaggaggaagttcaacaacggcgagatcaacttcgcggccgactgataa

SEQ ID NO: 56 - DNA, 2832 bp, Artificialsequence
  CD52_T02-R TALEN
atgggcgatcctaaaaagaaacgtaaggtcatcgataaggagaccgccgctgccaagttcgagagacagcacatggacagcatcgatatcgccgatctacgcacgctcggctacagccagcagcaacaggagaagatcaaaccgaaggttcgttcgacagtggcgcagcaccacgaggcactggtcggccacgggtttacacacgcgcacatcgttgcgttaagccaacacccggcagcgttagggaccgtcgctgtcaagtatcaggacatgatcgcagcgttgccagaggcgacacacgaagcgatcgttggcgtcggcaaacagtggtccggcgcacgcgctctggaggccttgctcacggtggcgggagagttgagaggtccaccgttacagttggacacaggccaacttctcaagattgcaaaacgtggcggcgtgaccgcagtggaggcagtgcatgcatggcgcaatgcactgacgggtgccccgctcaacttgaccccccagcaggtggtggccatcgccagcaatggcggtggcaagcaggcgctggagacggtccagcggctgttgccggtgctgtgccaggcccacggcttgaccccccagcaggtggtggccatcgccagcaataatggtggcaagcaggcgctggagacggtccagcggctgttgccggtgctgtgccaggcccacggcttgaccccggagcaggtggtggccatcgccagccacgatggcggcaagcaggcgctggagacggtccagcggctgttgccggtgctgtgccaggcccacggcttgaccccccagcaggtggtggccatcgccagcaatggcggtggcaagcaggcgctggagacggtccagcggctgttgccggtgctgtgccaggcccacggcttgaccccggagcaggtggtggccatcgccagccacgatggcggcaagcaggcgctggagacggtccagcggctgttgccggtgctgtgccaggcccacggcttgaccccccagcaggtggtggccatcgccagcaatggcggtggcaagcaggcgctggagacggtccagcggctgttgccggtgctgtgccaggcccacggcttgaccccccagcaggtggtggccatcgccagcaatggcggtggcaagcaggcgctggagacggtccagcggctgttgccggtgctgtgccaggcccacggcttgaccccggagcaggtggtggccatcgccagcaatattggtggcaagcaggcgctggagacggtgcaggcgctgttgccggtgctgtgccaggcccacggcttgaccccggagcaggtggtggccatcgccagccacgatggcggcaagcaggcgctggagacggtccagcggctgttgccggtgctgtgccaggcccacggcttgaccccggagcaggtggtggccatcgccagccacgatggcggcaagcaggcgctggagacggtccagcggctgttgccggtgctgtgccaggcccacggcttgaccccccagcaggtggtggccatcgccagcaatggcggtggcaagcaggcgctggagacggtccagcggctgttgccggtgctgtgccaggcccacggcttgaccccccagcaggtggtggccatcgccagcaataatggtggcaagcaggcgctggagacggtccagcggctgttgccggtgctgtgccaggcccacggcttgaccccccagcaggtggtggccatcgccagcaatggcggtggcaagcaggcgctggagacggtccagcggctgttgccggtgctgtgccaggcccacggcttgaccccggagcaggtggtggccatcgccagcaatattggtggcaagcaggcgctggagacggtgcaggcgctgttgccggtgctgtgccaggcccacggcttgaccccggagcaggtggtggccatcgccagccacgatggcggcaagcaggcgctggagacggtccagcggctgttgccggtgctgtgccaggcccacggcttgacccctcagcaggtggtggccatcgccagcaatggcggcggcaggccggcgctggagagcattgttgcccagttatctcgccctgatccggcgttggccgcgttgaccaacgaccacctcgtcgccttggcctgcctcggcgggcgtcctgcgctggatgcagtgaaaaagggattgggggatcctatcagccgttcccagctggtgaagtccgagctggaggagaagaaatccgagttgaggcacaagctgaagtacgtgccccacgagtacatcgagctgatcgagatcgcccggaacagcacccaggaccgtatcctggagatgaaggtgatggagttcttcatgaaggtgtacggctacaggggcaagcacctgggcggctccaggaagcccgacggcgccatctacaccgtgggctcccccatcgactacggcgtgatcgtggacaccaaggcctactccggcggctacaacctgcccatcggccaggccgacgaaatgcagaggtacgtggaggagaaccagaccaggaacaagcacatcaaccccaacgagtggtggaaggtgtacccctccagcgtgaccgagttcaagttcctgttcgtgtccggccacttcaagggcaactacaaggcccagctgaccaggctgaaccacatcaccaactgcaacggcgccgtgctgtccgtggaggagctcctgatcggcggcgagatgatcaaggccggcaccctgaccctggaggaggtgaggaggaagttcaacaacggcgagatcaacttcgcggccgactgataa

SEQ ID NO: 57 - DNA, 49 bp, Artificialsequence
  TRAC_T02
tttagaaagttcctgtgatgtcaagctggtcgagaaaagctttgaaaca

SEQ ID NO: 58 - DNA, 49 bp, Artificialsequence
  TRAC_T03
tccagtgacaagtctgtctgcctattcaccgattttgattctcaaacaa

SEQ ID NO: 59 - DNA, 49 bp, Artificialsequence
  TRAC_T04
tatatcacagacaaaactgtgctagacatgaggtctatggacttcaaga

SEQ ID NO: 60 - DNA, 49 bp, Artificialsequence
  TRAC_T05
tgaggtctatggacttcaagagcaacagtgctgtggcctggagcaacaa

SEQ ID NO: 61 - DNA, 47 bp, Artificial sequence
  CD52_T01
ttcctcttcctcctaccaccatcagcctcctttacctgtaccataac

SEQ ID NO: 62 - DNA, 43 bp, Artificial sequence
  CD52_T04
ttcctcctactcaccacagcctcctggtcttacctgtaccata

SEQ ID NO: 63 - DNA, 43 bp, Artificial sequence
  CD52_T05
tcctactcaccatcagctcctggttatttgctcttacctgtac

SEQ ID NO: 64 - DNA, 47 bp, Artificial sequence
  CD52_T06
ttatcccacttctcctctacagatacaaactttttgtcctgagagtc

SEQ ID NO: 65 - DNA, 47 bp, Artificial sequence
  CD52_T07
tggactctcaggacaaacgacaccagccaaatgctgaggggctgctg

SEQ ID NO: 66 - DNA, 60 bp, Artificial sequence
  Forward primer CD52
  misc_feature (31); (32); (33); (34); (35); (36); (37); (38); (39); (40): n is a or c or t or g
ccatctcatccctgcgtgtctccgactcagnnnnnnnnnncagatctgcagaaaggaagc

SEQ ID NO: 67 - DNA, 61 bp, Artificial sequence
  Forward primer TRAC
  misc_feature (31); (32); (33); (34); (35); (36); (37); (38); (39); (40): n is a or c or t or g
ccatctcatccctgcgtgtctccgactcagnnnnnnnnnnatcactggcatctggactcca

SEQ ID NO: 68 - DNA, 62 bp, Artificial sequence
  Forward primer TRBC1
  misc_feature (31); (32); (33); (34); (35); (36); (37); (38); (39); (40): n is a or c or t or g
ccatctcatccctgcgtgtctccgactcagnnnnnnnnnnagagcccctaccagaaccagac

SEQ ID NO: 69 - DNA, 62 bp, Artificial sequence
  Forward primer TRBC2
  misc_feature (31); (32); (33); (34); (35); (36); (37); (38); (39); (40): n is a or c or t or g
ccatctcatccctgcgtgtctccgactcagnnnnnnnnnnggacctagtaacataattgtgc

SEQ ID NO: 70 - DNA, 51 bp, Artificial sequence
  Reverse primer GR CD52
cctatcccctgtgtgccttggcagtctcagcctgttggagtccatctgctg

SEQ ID NO: 71 - DNA, 50 bp, Artificial sequence
  Reverse primer GR TRAC
cctatcccctgtgtgccttggcagtctcagcctcatgtctagcacagttt

SEQ ID NO: 72 - DNA, 51 bp, Artificial sequence
  Reverse primer GR TRBC1-2
cctatcccctgtgtgccttggcagtctcagaccagctcagctccacgtggt

SEQ ID NO: 73 - protein, 495 aa, Artificial sequence
  anti-CD19 CAR
METDTLLLWVLLLWVPGSTGEVQLQQSGPELIKPGASVKMSCKASGYTFTSYVMHWVKQKPGQGLEWIGYINPYNDGTKYNEKFKGKATLTSDKSSSTAYMELSSLTSEDSAVYYCARGTYYYGSRVFDYWGQGTTLTVSSGGGGSGGGGSGGGGSDIVMTQAAPSIPVTPGESVSISCRSSKSLLNSNGNTYLYWFLQRPGQSPQLLIYRMSNLASGVPDRFSGSGSGTAFTLRISRVEAEDVGVYYCMQHLEYPFTFGAGTKLELKRSDPTTTPAPRPPTPAPTIASQPLSLRPEACRPAAGGAVHTRGLDFACDIYIWAPLAGTCGVLLLSLVITLYCKRGRKKLLYIFKQPFMRPVQTTQEEDGCSCRFPEEEEGGCELRVKFSRSADAPAYQQGQNQLYNELNLGRREEYDVLDKRRGRDPEMGGKPRRKNPQEGLYNELQKDKMAEAYSEIGMKGERRRGKGHDGLYQGLSTATKDTYDALHMQALPPR

SEQ ID NO: 74 - DNA, 49 bp, Artificial sequence
  CTLA4_T01
tggccctgcactctcctgttttttcttctcttcatccctgtcttctgca

SEQ ID NO: 75 - DNA, 49 bp, Artificial sequence
  CTLA4_T03
ttttccatgctagcaatgcacgtggcccagcctgctgtggtactggcca

SEQ ID NO: 76 - DNA, 49 bp, Artificial sequence
  CTLA4_T04
tccatgctagcaatgcacgtggcccagcctgctgtggtactggccagca

SEQ ID NO: 77 - DNA, 49 bp, Artificial sequence
  PDCD1_T01
ttctccccagccctgctcgtggtgaccgaaggggacaacgccaccttca

SEQ ID NO: 78 - DNA, 49 bp, Artificial sequence
  PDCD1_T03
tacctctgtggggccatctccctggcccccaaggcgcagatcaaagaga

SEQ ID NO: 79 - protein, 530 aa, Artificial sequence
  Repeat CTLA4_T01-L
LTPQQVVAIASNNGGKQALETVQRLLPVLCQAHGLTPQQVVAIASNNGGKQALETVQRLLPVLCQAHGLTPEQVVAIASHDGGKQALETVQRLLPVLCQAHGLTPEQVVAIASHDGGKQALETVQRLLPVLCQAHGLTPEQVVAIASHDGGKQALETVQRLLPVLCQAHGLTPQQVVAIASNGGGKQALETVQRLLPVLCQAHGLTPQQVVAIASNNGGKQALETVQRLLPVLCQAHGLTPEQVVAIASHDGGKQALETVQRLLPVLCQAHGLTPEQVVAIASNIGGKQALETVQALLPVLCQAHGLTPEQVVAIASHDGGKQALETVQRLLPVLCQAHGLTPQQVVAIASNGGGKQALETVQRLLPVLCQAHGLTPEQVVAIASHDGGKQALETVQRLLPVLCQAHGLTPQQVVAIASNGGGKQALETVQRLLPVLCQAHGLTPEQVVAIASHDGGKQALETVQRLLPVLCQAHGLTPEQVVAIASHDGGKQALETVQRLLPVLCQAHGLTPQQVVAIASNGGGRPALE

SEQ ID NO: 80 - protein, 530 aa, Artificial sequence
  Repeat CTLA4_T01-R
LTPQQVVAIASNNGGKQALETVQRLLPVLCQAHGLTPEQVVAIASHDGGKQALETVQRLLPVLCQAHGLTPEQVVAIASNIGGKQALETVQALLPVLCQAHGLTPQQVVAIASNNGGKQALETVQRLLPVLCQAHGLTPEQVVAIASNIGGKQALETVQALLPVLCQAHGLTPEQVVAIASNIGGKQALETVQALLPVLCQAHGLTPQQVVAIASNNGGKQALETVQRLLPVLCQAHGLTPEQVVAIASNIGGKQALETVQALLPVLCQAHGLTPEQVVAIASHDGGKQALETVQRLLPVLCQAHGLTPEQVVAIASNIGGKQALETVQALLPVLCQAHGLTPQQVVAIASNNGGKQALETVQRLLPVLCQAHGLTPQQVVAIASNNGGKQALETVQRLLPVLCQAHGLTPQQVVAIASNNGGKQALETVQRLLPVLCQAHGLTPEQVVAIASNIGGKQALETVQALLPVLCQAHGLTPQQVVAIASNGGGKQALETVQRLLPVLCQAHGLTPQQVVAIASNGGGRPALE

SEQ ID NO: 81 - protein, 530 aa, Artificial sequence
  RepeatCTLA4_T03-L
LTPQQVVAIASNGGGKQALETVQRLLPVLCQAHGLTPQQVVAIASNGGGKQALETVQRLLPVLCQAHGLTPQQVVAIASNGGGKQALETVQRLLPVLCQAHGLTPEQVVAIASHDGGKQALETVQRLLPVLCQAHGLTPEQVVAIASHDGGKQALETVQRLLPVLCQAHGLTPEQVVAIASNIGGKQALETVQALLPVLCQAHGLTPQQVVAIASNGGGKQALETVQRLLPVLCQAHGLTPQQVVAIASNNGGKQALETVQRLLPVLCQAHGLTPEQVVAIASHDGGKQALETVQRLLPVLCQAHGLTPQQVVAIASNGGGKQALETVQRLLPVLCQAHGLTPEQVVAIASNIGGKQALETVQALLPVLCQAHGLTPQQVVAIASNNGGKQALETVQRLLPVLCQAHGLTPEQVVAIASHDGGKQALETVQRLLPVLCQAHGLTPEQVVAIASNIGGKQALETVQALLPVLCQAHGLTPEQVVAIASNIGGKQALETVQALLPVLCQAHGLTPQQVVAIASNGGGRPALE

SEQ ID NO: 82 - protein, 530 aa, Artificial sequence
  Repeat CTLA4_T03-R
LTPQQVVAIASNNGGKQALETVQRLLPVLCQAHGLTPQQVVAIASNNGGKQALETVQRLLPVLCQAHGLTPEQVVAIASHDGGKQALETVQRLLPVLCQAHGLTPEQVVAIASHDGGKQALETVQRLLPVLCQAHGLTPEQVVAIASNIGGKQALETVQALLPVLCQAHGLTPQQVVAIASNNGGKQALETVQRLLPVLCQAHGLTPQQVVAIASNGGGKQALETVQRLLPVLCQAHGLTPEQVVAIASNIGGKQALETVQALLPVLCQAHGLTPEQVVAIASHDGGKQALETVQRLLPVLCQAHGLTPEQVVAIASHDGGKQALETVQRLLPVLCQAHGLTPEQVVAIASNIGGKQALETVQALLPVLCQAHGLTPEQVVAIASHDGGKQALETVQRLLPVLCQAHGLTPEQVVAIASNIGGKQALETVQALLPVLCQAHGLTPQQVVAIASNNGGKQALETVQRLLPVLCQAHGLTPEQVVAIASHDGGKQALETVQRLLPVLCQAHGLTPQQVVAIASNGGGRPALE

SEQ ID NO: 83 - protein, 530 aa, Artificial sequence
  Repeat CTLA4_T04-L
LTPEQVVAIASHDGGKQALETVQRLLPVLCQAHGLTPEQVVAIASHDGGKQALETVQRLLPVLCQAHGLTPEQVVAIASNIGGKQALETVQALLPVLCQAHGLTPQQVVAIASNGGGKQALETVQRLLPVLCQAHGLTPQQVVAIASNNGGKQALETVQRLLPVLCQAHGLTPEQVVAIASHDGGKQALETVQRLLPVLCQAHGLTPQQVVAIASNGGGKQALETVQRLLPVLCQAHGLTPEQVVAIASNIGGKQALETVQALLPVLCQAHGLTPQQVVAIASNNGGKQALETVQRLLPVLCQAHGLTPEQVVAIASHDGGKQALETVQRLLPVLCQAHGLTPEQVVAIASNIGGKQALETVQALLPVLCQAHGLTPEQVVAIASNIGGKQALETVQALLPVLCQAHGLTPQQVVAIASNGGGKQALETVQRLLPVLCQAHGLTPQQVVAIASNNGGKQALETVQRLLPVLCQAHGLTPEQVVAIASHDGGKQALETVQRLLPVLCQAHGLTPQQVVAIASNGGGRPALE

SEQ ID NO: 84 - protein, 530 aa, Artificial sequence
  Repeat CTLA4_T04-R
LTPQQVVAIASNNGGKQALETVQRLLPVLCQAHGLTPEQVVAIASHDGGKQALETVQRLLPVLCQAHGLTPQQVVAIASNGGGKQALETVQRLLPVLCQAHGLTPQQVVAIASNNGGKQALETVQRLLPVLCQAHGLTPQQVVAIASNNGGKQALETVQRLLPVLCQAHGLTPEQVVAIASHDGGKQALETVQRLLPVLCQAHGLTPEQVVAIASHDGGKQALETVQRLLPVLCQAHGLTPEQVVAIASNIGGKQALETVQALLPVLCQAHGLTPQQVVAIASNNGGKQALETVQRLLPVLCQAHGLTPQQVVAIASNGGGKQALETVQRLLPVLCQAHGLTPEQVVAIASNIGGKQALETVQALLPVLCQAHGLTPEQVVAIASHDGGKQALETVQRLLPVLCQAHGLTPEQVVAIASHDGGKQALETVQRLLPVLCQAHGLTPEQVVAIASNIGGKQALETVQALLPVLCQAHGLTPEQVVAIASHDGGKQALETVQRLLPVLCQAHGLTPQQVVAIASNGGGRPALE

SEQ ID NO: 85 - protein, 530 aa, Artificial sequence
  Repeat PDCD1_T01-L
LTPQQVVAIASNGGGKQALETVQRLLPVLCQAHGLTPEQVVAIASHDGGKQALETVQRLLPVLCQAHGLTPQQVVAIASNGGGKQALETVQRLLPVLCQAHGLTPEQVVAIASHDGGKQALETVQRLLPVLCQAHGLTPEQVVAIASHDGGKQALETVQRLLPVLCQAHGLTPEQVVAIASHDGGKQALETVQRLLPVLCQAHGLTPEQVVAIASHDGGKQALETVQRLLPVLCQAHGLTPEQVVAIASNIGGKQALETVQALLPVLCQAHGLTPQQVVAIASNNGGKQALETVQRLLPVLCQAHGLTPEQVVAIASHDGGKQALETVQRLLPVLCQAHGLTPEQVVAIASHDGGKQALETVQRLLPVLCQAHGLTPEQVVAIASHDGGKQALETVQRLLPVLCQAHGLTPQQVVAIASNGGGKQALETVQRLLPVLCQAHGLTPQQVVAIASNNGGKQALETVQRLLPVLCQAHGLTPEQVVAIASHDGGKQALETVQRLLPVLCQAHGLTPQQVVAIASNGGGRPALE

SEQ ID NO: 86 - protein, 529 aa, Artificial sequence
  RepeatPDCD1_T01-R
LTPQQVVAIASNNGGKQALETVQRLLPVLCQAHGLTPEQVVAIASNIGGKQALETVQALLPVLCQAHGLTPEQVVAIASNIGGKQALETVQALLPVLCQAHGLTPQQVVAIASNNGGKQALETVQRLLPVLCQAHGLTPQQVVAIASNNGGKQALETVQRLLPVLCQAHGLTPQQVVAIASNGGGKQALETVQRLLPVLCQAHGLTPQQVVAIASNNGGKQALETVQRLLPVLCQAHGLTPQQVVAIASNNGGKQALETVQRLLPVLCQAHGLTPEQVVAIASNGGKQALETVQRLLPVLCQAHGLTPQQVVAIASNNGGKQALETVQRLLPVLCQAHGLTPQQVVAIASNGGGKQALETVQRLLPVLCQAHGLTPQQVVAIASNGGGKQALETVQRLLPVLCQAHGLTPQQVVAIASNNGGKQALETVQRLLPVLCQAHGLTPQQVVAIASNGGGKQALETVQRLLPVLCQAHGLTPEQVVAIASHDGGKQALETVQRLLPVLCQAHGLTPQQVVAIASNGGGRPALE

SEQ ID NO: 87 - protein, 530 aa, Artificial sequence
  Repeat PDCD1_T03-L
LTPEQVVAIASNIGGKQALETVQALLPVLCQAHGLTPEQVVAIASHDGGKQALETVQRLLPVLCQAHGLTPEQVVAIASHDGGKQALETVQRLLPVLCQAHGLTPQQVVAIASNGGGKQALETVQRLLPVLCQAHGLTPEQVVAIASHDGGKQALETVQRLLPVLCQAHGLTPQQVVAIASNGGGKQALETVQRLLPVLCQAHGLTPQQVVAIASNNGGKQALETVQRLLPVLCQAHGLTPQQVVAIASNGGGKQALETVQRLLPVLCQAHGLTPQQVVAIASNNGGKQALETVQRLLPVLCQAHGLTPQQVVAIASNNGGKQALETVQRLLPVLCQAHGLTPQQVVAIASNNGGKQALETVQRLLPVLCQAHGLTPQQVVAIASNNGGKQALETVQRLLPVLCQAHGLTPEQVVAIASHDGGKQALETVQRLLPVLCQAHGLTPEQVVAIASHDGGKQALETVQRLLPVLCQAHGLTPEQVVAIASNIGGKQALETVQALLPVLCQAHGLTPQQVVAIASNGGGRPALE

SEQ ID NO: 88 - protein, 529 aa, Artificial sequence
  Repeat PDCD1_T03-R
LTPEQVVAIASHDGGKQALETVQRLLPVLCQAHGLTPQQVVAIASNGGGKQALETVQRLLPVLCQAHGLTPEQVVAIASHDGGKQALETVQRLLPVLCQAHGLTPQQVVAIASNGGGKQALETVQRLLPVLCQAHGLTPQQVVAIASNGGGKQALETVQRLLPVLCQAHGLTPQQVVAIASNGGGKQALETVQRLLPVLCQAHGLTPQQVVAIASNNGGKQALETVQRLLPVLCQAHGLTPEQVVAIASNIGGKQALETVQALLPVLCQAHGLTPQQVVAIASNGGGKQALETVQRLLPVLCQAHGLTPEQVVAIASHDGGKQALETVQRLLPVLCQAHGLTPQQVVAIASNGGGKQALETVQRLLPVLCQAHGLTPQQVVAIASNNGGKQALETVQRLLPVLCQAHGLTPEQVVAIASNGGKQALETVQRLLPVLCQAHGLTPQQVVAIASNNGGKQALETVQRLLPVLCQAHGLTPEQVVAIASHDGGKQALETVQRLLPVLCQAHGLTPQQVVAIASNGGGRPALE

SEQ ID NO: 89 - DNA, 2814 bp, Artificial sequence
  CTLA4_T01-L  TALEN
atgggcgatcctaaaaagaaacgtaaggtcatcgattacccatacgatgttccagattacgctatcgatatcgccgatctacgcacgctcggctacagccagcagcaacaggagaagatcaaaccgaaggttcgttcgacagtggcgcagcaccacgaggcactggtcggccacgggtttacacacgcgcacatcgttgcgttaagccaacacccggcagcgttagggaccgtcgctgtcaagtatcaggacatgatcgcagcgttgccagaggcgacacacgaagcgatcgttggcgtcggcaaacagtggtccggcgcacgcgctctggaggccttgctcacggtggcgggagagttgagaggtccaccgttacagttggacacaggccaacttctcaagattgcaaaacgtggcggcgtgaccgcagtggaggcagtgcatgcatggcgcaatgcactgacgggtgccccgctcaacttgaccccccagcaggtggtggccatcgccagcaataatggtggcaagcaggcgctggagacggtccagcggctgttgccggtgctgtgccaggcccacggcttgaccccccagcaggtggtggccatcgccagcaataatggtggcaagcaggcgctggagacggtccagcggctgttgccggtgctgtgccaggcccacggcttgaccccggagcaggtggtggccatcgccagccacgatggcggcaagcaggcgctggagacggtccagcggctgttgccggtgctgtgccaggcccacggcttgaccccggagcaggtggtggccatcgccagccacgatggcggcaagcaggcgctggagacggtccagcggctgttgccggtgctgtgccaggcccacggcttgaccccggagcaggtggtggccatcgccagccacgatggcggcaagcaggcgctggagacggtccagcggctgttgccggtgctgtgccaggcccacggcttgaccccccagcaggtggtggccatcgccagcaatggcggtggcaagcaggcgctggagacggtccagcggctgttgccggtgctgtgccaggcccacggcttgaccccccagcaggtggtggccatcgccagcaataatggtggcaagcaggcgctggagacggtccagcggctgttgccggtgctgtgccaggcccacggcttgaccccggagcaggtggtggccatcgccagccacgatggcggcaagcaggcgctggagacggtccagcggctgttgccggtgctgtgccaggcccacggcttgaccccggagcaggtggtggccatcgccagcaatattggtggcaagcaggcgctggagacggtgcaggcgctgttgccggtgctgtgccaggcccacggcttgaccccggagcaggtggtggccatcgccagccacgatggcggcaagcaggcgctggagacggtccagcggctgttgccggtgctgtgccaggcccacggcttgaccccccagcaggtggtggccatcgccagcaatggcggtggcaagcaggcgctggagacggtccagcggctgttgccggtgctgtgccaggcccacggcttgaccccggagcaggtggtggccatcgccagccacgatggcggcaagcaggcgctggagacggtccagcggctgttgccggtgctgtgccaggcccacggcttgaccccccagcaggtggtggccatcgccagcaatggcggtggcaagcaggcgctggagacggtccagcggctgttgccggtgctgtgccaggcccacggcttgaccccggagcaggtggtggccatcgccagccacgatggcggcaagcaggcgctggagacggtccagcggctgttgccggtgctgtgccaggcccacggcttgaccccggagcaggtggtggccatcgccagccacgatggcggcaagcaggcgctggagacggtccagcggctgttgccggtgctgtgccaggcccacggcttgacccctcagcaggtggtggccatcgccagcaatggcggcggcaggccggcgctggagagcattgttgcccagttatctcgccctgatccggcgttggccgcgttgaccaacgaccacctcgtcgccttggcctgcctcggcgggcgtcctgcgctggatgcagtgaaaaagggattgggggatcctatcagccgttcccagctggtgaagtccgagctggaggagaagaaatccgagttgaggcacaagctgaagtacgtgccccacgagtacatcgagctgatcgagatcgcccggaacagcacccaggaccgtatcctggagatgaaggtgatggagttcttcatgaaggtgtacggctacaggggcaagcacctgggcggctccaggaagcccgacggcgccatctacaccgtgggctcccccatcgactacggcgtgatcgtggacaccaaggcctactccggcggctacaacctgcccatcggccaggccgacgaaatgcagaggtacgtggaggagaaccagaccaggaacaagcacatcaaccccaacgagtggtggaaggtgtacccctccagcgtgaccgagttcaagttcctgttcgtgtccggccacttcaagggcaactacaaggcccagctgaccaggctgaaccacatcaccaactgcaacggcgccgtgctgtccgtggaggagctcctgatcggcggcgagatgatcaaggccggcaccctgaccctggaggaggtgaggaggaagttcaacaacggcgagatcaacttcgcggccgactgataa

SEQ ID NO: 90 - DNA, 2832 bp, Artificial sequence
  CTLA4_T01-R TALEN
atgggcgatcctaaaaagaaacgtaaggtcatcgataaggagaccgccgctgccaagttcgagagacagcacatggacagcatcgatatcgccgatctacgcacgctcggctacagccagcagcaacaggagaagatcaaaccgaaggttcgttcgacagtggcgcagcaccacgaggcactggtcggccacgggtttacacacgcgcacatcgttgcgttaagccaacacccggcagcgttagggaccgtcgctgtcaagtatcaggacatgatcgcagcgttgccagaggcgacacacgaagcgatcgttggcgtcggcaaacagtggtccggcgcacgcgctctggaggccttgctcacggtggcgggagagttgagaggtccaccgttacagttggacacaggccaacttctcaagattgcaaaacgtggcggcgtgaccgcagtggaggcagtgcatgcatggcgcaatgcactgacgggtgccccgctcaacttgaccccccagcaggtggtggccatcgccagcaataatggtggcaagcaggcgctggagacggtccagcggctgttgccggtgctgtgccaggcccacggcttgaccccggagcaggtggtggccatcgccagccacgatggcggcaagcaggcgctggagacggtccagcggctgttgccggtgctgtgccaggcccacggcttgaccccggagcaggtggtggccatcgccagcaatattggtggcaagcaggcgctggagacggtgcaggcgctgttgccggtgctgtgccaggcccacggcttgaccccccagcaggtggtggccatcgccagcaataatggtggcaagcaggcgctggagacggtccagcggctgttgccggtgctgtgccaggcccacggcttgaccccggagcaggtggtggccatcgccagcaatattggtggcaagcaggcgctggagacggtgcaggcgctgttgccggtgctgtgccaggcccacggcttgaccccggagcaggtggtggccatcgccagcaatattggtggcaagcaggcgctggagacggtgcaggcgctgttgccggtgctgtgccaggcccacggcttgaccccccagcaggtggtggccatcgccagcaataatggtggcaagcaggcgctggagacggtccagcggctgttgccggtgctgtgccaggcccacggcttgaccccggagcaggtggtggccatcgccagcaatattggtggcaagcaggcgctggagacggtgcaggcgctgttgccggtgctgtgccaggcccacggcttgaccccggagcaggtggtggccatcgccagccacgatggcggcaagcaggcgctggagacggtccagcggctgttgccggtgctgtgccaggcccacggcttgaccccggagcaggtggtggccatcgccagcaatattggtggcaagcaggcgctggagacggtgcaggcgctgttgccggtgctgtgccaggcccacggcttgaccccccagcaggtggtggccatcgccagcaataatggtggcaagcaggcgctggagacggtccagcggctgttgccggtgctgtgccaggcccacggcttgaccccccagcaggtggtggccatcgccagcaataatggtggcaagcaggcgctggagacggtccagcggctgttgccggtgctgtgccaggcccacggcttgaccccccagcaggtggtggccatcgccagcaataatggtggcaagcaggcgctggagacggtccagcggctgttgccggtgctgtgccaggcccacggcttgaccccggagcaggtggtggccatcgccagcaatattggtggcaagcaggcgctggagacggtgcaggcgctgttgccggtgctgtgccaggcccacggcttgaccccccagcaggtggtggccatcgccagcaatggcggtggcaagcaggcgctggagacggtccagcggctgttgccggtgctgtgccaggcccacggcttgacccctcagcaggtggtggccatcgccagcaatggcggcggcaggccggcgctggagagcattgttgcccagttatctcgccctgatccggcgttggccgcgttgaccaacgaccacctcgtcgccttggcctgcctcggcgggcgtcctgcgctggatgcagtgaaaaagggattgggggatcctatcagccgttcccagctggtgaagtccgagctggaggagaagaaatccgagttgaggcacaagctgaagtacgtgccccacgagtacatcgagctgatcgagatcgcccggaacagcacccaggaccgtatcctggagatgaaggtgatggagttcttcatgaaggtgtacggctacaggggcaagcacctgggcggctccaggaagcccgacggcgccatctacaccgtgggctcccccatcgactacggcgtgatcgtggacaccaaggcctactccggcggctacaacctgcccatcggccaggccgacgaaatgcagaggtacgtggaggagaaccagaccaggaacaagcacatcaaccccaacgagtggtggaaggtgtacccctccagcgtgaccgagttcaagttcctgttcgtgtccggccacttcaagggcaactacaaggcccagctgaccaggctgaaccacatcaccaactgcaacggcgccgtgctgtccgtggaggagctcctgatcggcggcgagatgatcaaggccggcaccctgaccctggaggaggtgaggaggaagttcaacaacggcgagatcaacttcgcggccgactgataa

SEQ ID NO: 91 - DNA, 2814 bp, Artificial sequence
  CTLA4_T03-L TALEN
atgggcgatcctaaaaagaaacgtaaggtcatcgattacccatacgatgttccagattacgctatcgatatcgccgatctacgcacgctcggctacagccagcagcaacaggagaagatcaaaccgaaggttcgttcgacagtggcgcagcaccacgaggcactggtcggccacgggtttacacacgcgcacatcgttgcgttaagccaacacccggcagcgttagggaccgtcgctgtcaagtatcaggacatgatcgcagcgttgccagaggcgacacacgaagcgatcgttggcgtcggcaaacagtggtccggcgcacgcgctctggaggccttgctcacggtggcgggagagttgagaggtccaccgttacagttggacacaggccaacttctcaagattgcaaaacgtggcggcgtgaccgcagtggaggcagtgcatgcatggcgcaatgcactgacgggtgccccgctcaacttgaccccccagcaggtggtggccatcgccagcaatggcggtggcaagcaggcgctggagacggtccagcggctgttgccggtgctgtgccaggcccacggcttgaccccccagcaggtggtggccatcgccagcaatggcggtggcaagcaggcgctggagacggtccagcggctgttgccggtgctgtgccaggcccacggcttgaccccccagcaggtggtggccatcgccagcaatggcggtggcaagcaggcgctggagacggtccagcggctgttgccggtgctgtgccaggcccacggcttgaccccggagcaggtggtggccatcgccagccacgatggcggcaagcaggcgctggagacggtccagcggctgttgccggtgctgtgccaggcccacggcttgaccccggagcaggtggtggccatcgccagccacgatggcggcaagcaggcgctggagacggtccagcggctgttgccggtgctgtgccaggcccacggcttgaccccggagcaggtggtggccatcgccagcaatattggtggcaagcaggcgctggagacggtgcaggcgctgttgccggtgctgtgccaggcccacggcttgaccccccagcaggtggtggccatcgccagcaatggcggtggcaagcaggcgctggagacggtccagcggctgttgccggtgctgtgccaggcccacggcttgaccccccagcaggtggtggccatcgccagcaataatggtggcaagcaggcgctggagacggtccagcggctgttgccggtgctgtgccaggcccacggcttgaccccggagcaggtggtggccatcgccagccacgatggcggcaagcaggcgctggagacggtccagcggctgttgccggtgctgtgccaggcccacggcttgaccccccagcaggtggtggccatcgccagcaatggcggtggcaagcaggcgctggagacggtccagcggctgttgccggtgctgtgccaggcccacggcttgaccccggagcaggtggtggccatcgccagcaatattggtggcaagcaggcgctggagacggtgcaggcgctgttgccggtgctgtgccaggcccacggcttgaccccccagcaggtggtggccatcgccagcaataatggtggcaagcaggcgctggagacggtccagcggctgttgccggtgctgtgccaggcccacggcttgaccccggagcaggtggtggccatcgccagccacgatggcggcaagcaggcgctggagacggtccagcggctgttgccggtgctgtgccaggcccacggcttgaccccggagcaggtggtggccatcgccagcaatattggtggcaagcaggcgctggagacggtgcaggcgctgttgccggtgctgtgccaggcccacggcttgaccccggagcaggtggtggccatcgccagcaatattggtggcaagcaggcgctggagacggtgcaggcgctgttgccggtgctgtgccaggcccacggcttgacccctcagcaggtggtggccatcgccagcaatggcggcggcaggccggcgctggagagcattgttgcccagttatctcgccctgatccggcgttggccgcgttgaccaacgaccacctcgtcgccttggcctgcctcggcgggcgtcctgcgctggatgcagtgaaaaagggattgggggatcctatcagccgttcccagctggtgaagtccgagctggaggagaagaaatccgagttgaggcacaagctgaagtacgtgccccacgagtacatcgagctgatcgagatcgcccggaacagcacccaggaccgtatcctggagatgaaggtgatggagttcttcatgaaggtgtacggctacaggggcaagcacctgggcggctccaggaagcccgacggcgccatctacaccgtgggctcccccatcgactacggcgtgatcgtggacaccaaggcctactccggcggctacaacctgcccatcggccaggccgacgaaatgcagaggtacgtggaggagaaccagaccaggaacaagcacatcaaccccaacgagtggtggaaggtgtacccctccagcgtgaccgagttcaagttcctgttcgtgtccggccacttcaagggcaactacaaggcccagctgaccaggctgaaccacatcaccaactgcaacggcgccgtgctgtccgtggaggagctcctgatcggcggcgagatgatcaaggccggcaccctgaccctggaggaggtgaggaggaagttcaacaacggcgagatcaacttcgcggccgactgataa

SEQ ID NO: 92 - DNA, 2832 bp, Artificial sequence
  CTLA4_T03-RTALEN
atgggcgatcctaaaaagaaacgtaaggtcatcgataaggagaccgccgctgccaagttcgagagacagcacatggacagcatcgatatcgccgatctacgcacgctcggctacagccagcagcaacaggagaagatcaaaccgaaggttcgttcgacagtggcgcagcaccacgaggcactggtcggccacgggtttacacacgcgcacatcgttgcgttaagccaacacccggcagcgttagggaccgtcgctgtcaagtatcaggacatgatcgcagcgttgccagaggcgacacacgaagcgatcgttggcgtcggcaaacagtggtccggcgcacgcgctctggaggccttgctcacggtggcgggagagttgagaggtccaccgttacagttggacacaggccaacttctcaagattgcaaaacgtggcggcgtgaccgcagtggaggcagtgcatgcatggcgcaatgcactgacgggtgccccgctcaacttgaccccccagcaggtggtggccatcgccagcaataatggtggcaagcaggcgctggagacggtccagcggctgttgccggtgctgtgccaggcccacggcttgaccccccagcaggtggtggccatcgccagcaataatggtggcaagcaggcgctggagacggtccagcggctgttgccggtgctgtgccaggcccacggcttgaccccggagcaggtggtggccatcgccagccacgatggcggcaagcaggcgctggagacggtccagcggctgttgccggtgctgtgccaggcccacggcttgaccccggagcaggtggtggccatcgccagccacgatggcggcaagcaggcgctggagacggtccagcggctgttgccggtgctgtgccaggcccacggcttgaccccggagcaggtggtggccatcgccagcaatattggtggcaagcaggcgctggagacggtgcaggcgctgttgccggtgctgtgccaggcccacggcttgaccccccagcaggtggtggccatcgccagcaataatggtggcaagcaggcgctggagacggtccagcggctgttgccggtgctgtgccaggcccacggcttgaccccccagcaggtggtggccatcgccagcaatggcggtggcaagcaggcgctggagacggtccagcggctgttgccggtgctgtgccaggcccacggcttgaccccggagcaggtggtggccatcgccagcaatattggtggcaagcaggcgctggagacggtgcaggcgctgttgccggtgctgtgccaggcccacggcttgaccccggagcaggtggtggccatcgccagccacgatggcggcaagcaggcgctggagacggtccagcggctgttgccggtgctgtgccaggcccacggcttgaccccggagcaggtggtggccatcgccagccacgatggcggcaagcaggcgctggagacggtccagcggctgttgccggtgctgtgccaggcccacggcttgaccccggagcaggtggtggccatcgccagcaatattggtggcaagcaggcgctggagacggtgcaggcgctgttgccggtgctgtgccaggcccacggcttgaccccggagcaggtggtggccatcgccagccacgatggcggcaagcaggcgctggagacggtccagcggctgttgccggtgctgtgccaggcccacggcttgaccccggagcaggtggtggccatcgccagcaatattggtggcaagcaggcgctggagacggtgcaggcgctgttgccggtgctgtgccaggcccacggcttgaccccccagcaggtggtggccatcgccagcaataatggtggcaagcaggcgctggagacggtccagcggctgttgccggtgctgtgccaggcccacggcttgaccccggagcaggtggtggccatcgccagccacgatggcggcaagcaggcgctggagacggtccagcggctgttgccggtgctgtgccaggcccacggcttgacccctcagcaggtggtggccatcgccagcaatggcggcggcaggccggcgctggagagcattgttgcccagttatctcgccctgatccggcgttggccgcgttgaccaacgaccacctcgtcgccttggcctgcctcggcgggcgtcctgcgctggatgcagtgaaaaagggattgggggatcctatcagccgttcccagctggtgaagtccgagctggaggagaagaaatccgagttgaggcacaagctgaagtacgtgccccacgagtacatcgagctgatcgagatcgcccggaacagcacccaggaccgtatcctggagatgaaggtgatggagttcttcatgaaggtgtacggctacaggggcaagcacctgggcggctccaggaagcccgacggcgccatctacaccgtgggctcccccatcgactacggcgtgatcgtggacaccaaggcctactccggcggctacaacctgcccatcggccaggccgacgaaatgcagaggtacgtggaggagaaccagaccaggaacaagcacatcaaccccaacgagtggtggaaggtgtacccctccagcgtgaccgagttcaagttcctgttcgtgtccggccacttcaagggcaactacaaggcccagctgaccaggctgaaccacatcaccaactgcaacggcgccgtgctgtccgtggaggagctcctgatcggcggcgagatgatcaaggccggcaccctgaccctggaggaggtgaggaggaagttcaacaacggcgagatcaacttcgcggccgactgataa

SEQ ID NO: 93 - DNA, 2814 bp, Artificial sequence
  CTLA4_T04-L TALEN
atgggcgatcctaaaaagaaacgtaaggtcatcgattacccatacgatgttccagattacgctatcgatatcgccgatctacgcacgctcggctacagccagcagcaacaggagaagatcaaaccgaaggttcgttcgacagtggcgcagcaccacgaggcactggtcggccacgggtttacacacgcgcacatcgttgcgttaagccaacacccggcagcgttagggaccgtcgctgtcaagtatcaggacatgatcgcagcgttgccagaggcgacacacgaagcgatcgttggcgtcggcaaacagtggtccggcgcacgcgctctggaggccttgctcacggtggcgggagagttgagaggtccaccgttacagttggacacaggccaacttctcaagattgcaaaacgtggcggcgtgaccgcagtggaggcagtgcatgcatggcgcaatgcactgacgggtgccccgctcaacttgaccccggagcaggtggtggccatcgccagccacgatggcggcaagcaggcgctggagacggtccagcggctgttgccggtgctgtgccaggcccacggcttgaccccggagcaggtggtggccatcgccagccacgatggcggcaagcaggcgctggagacggtccagcggctgttgccggtgctgtgccaggcccacggcttgaccccggagcaggtggtggccatcgccagcaatattggtggcaagcaggcgctggagacggtgcaggcgctgttgccggtgctgtgccaggcccacggcttgaccccccagcaggtggtggccatcgccagcaatggcggtggcaagcaggcgctggagacggtccagcggctgttgccggtgctgtgccaggcccacggcttgaccccccagcaggtggtggccatcgccagcaataatggtggcaagcaggcgctggagacggtccagcggctgttgccggtgctgtgccaggcccacggcttgaccccggagcaggtggtggccatcgccagccacgatggcggcaagcaggcgctggagacggtccagcggctgttgccggtgctgtgccaggcccacggcttgaccccccagcaggtggtggccatcgccagcaatggcggtggcaagcaggcgctggagacggtccagcggctgttgccggtgctgtgccaggcccacggcttgaccccggagcaggtggtggccatcgccagcaatattggtggcaagcaggcgctggagacggtgcaggcgctgttgccggtgctgtgccaggcccacggcttgaccccccagcaggtggtggccatcgccagcaataatggtggcaagcaggcgctggagacggtccagcggctgttgccggtgctgtgccaggcccacggcttgaccccggagcaggtggtggccatcgccagccacgatggcggcaagcaggcgctggagacggtccagcggctgttgccggtgctgtgccaggcccacggcttgaccccggagcaggtggtggccatcgccagcaatattggtggcaagcaggcgctggagacggtgcaggcgctgttgccggtgctgtgccaggcccacggcttgaccccggagcaggtggtggccatcgccagcaatattggtggcaagcaggcgctggagacggtgcaggcgctgttgccggtgctgtgccaggcccacggcttgaccccccagcaggtggtggccatcgccagcaatggcggtggcaagcaggcgctggagacggtccagcggctgttgccggtgctgtgccaggcccacggcttgaccccccagcaggtggtggccatcgccagcaataatggtggcaagcaggcgctggagacggtccagcggctgttgccggtgctgtgccaggcccacggcttgaccccggagcaggtggtggccatcgccagccacgatggcggcaagcaggcgctggagacggtccagcggctgttgccggtgctgtgccaggcccacggcttgacccctcagcaggtggtggccatcgccagcaatggcggcggcaggccggcgctggagagcattgttgcccagttatctcgccctgatccggcgttggccgcgttgaccaacgaccacctcgtcgccttggcctgcctcggcgggcgtcctgcgctggatgcagtgaaaaagggattgggggatcctatcagccgttcccagctggtgaagtccgagctggaggagaagaaatccgagttgaggcacaagctgaagtacgtgccccacgagtacatcgagctgatcgagatcgcccggaacagcacccaggaccgtatcctggagatgaaggtgatggagttcttcatgaaggtgtacggctacaggggcaagcacctgggcggctccaggaagcccgacggcgccatctacaccgtgggctcccccatcgactacggcgtgatcgtggacaccaaggcctactccggcggctacaacctgcccatcggccaggccgacgaaatgcagaggtacgtggaggagaaccagaccaggaacaagcacatcaaccccaacgagtggtggaaggtgtacccctccagcgtgaccgagttcaagttcctgttcgtgtccggccacttcaagggcaactacaaggcccagctgaccaggctgaaccacatcaccaactgcaacggcgccgtgctgtccgtggaggagctcctgatcggcggcgagatgatcaaggccggcaccctgaccctggaggaggtgaggaggaagttcaacaacggcgagatcaacttcgcggccgactgataa

SEQ ID NO: 94 - DNA, 2832 bp, Artificial sequence
  CTLA4_T04-R TALEN
atgggcgatcctaaaaagaaacgtaaggtcatcgataaggagaccgccgctgccaagttcgagagacagcacatggacagcatcgatatcgccgatctacgcacgctcggctacagccagcagcaacaggagaagatcaaaccgaaggttcgttcgacagtggcgcagcaccacgaggcactggtcggccacgggtttacacacgcgcacatcgttgcgttaagccaacacccggcagcgttagggaccgtcgctgtcaagtatcaggacatgatcgcagcgttgccagaggcgacacacgaagcgatcgttggcgtcggcaaacagtggtccggcgcacgcgctctggaggccttgctcacggtggcgggagagttgagaggtccaccgttacagttggacacaggccaacttctcaagattgcaaaacgtggcggcgtgaccgcagtggaggcagtgcatgcatggcgcaatgcactgacgggtgccccgctcaacttgaccccccagcaggtggtggccatcgccagcaataatggtggcaagcaggcgctggagacggtccagcggctgttgccggtgctgtgccaggcccacggcttgaccccggagcaggtggtggccatcgccagccacgatggcggcaagcaggcgctggagacggtccagcggctgttgccggtgctgtgccaggcccacggcttgaccccccagcaggtggtggccatcgccagcaatggcggtggcaagcaggcgctggagacggtccagcggctgttgccggtgctgtgccaggcccacggcttgaccccccagcaggtggtggccatcgccagcaataatggtggcaagcaggcgctggagacggtccagcggctgttgccggtgctgtgccaggcccacggcttgaccccccagcaggtggtggccatcgccagcaataatggtggcaagcaggcgctggagacggtccagcggctgttgccggtgctgtgccaggcccacggcttgaccccggagcaggtggtggccatcgccagccacgatggcggcaagcaggcgctggagacggtccagcggctgttgccggtgctgtgccaggcccacggcttgaccccggagcaggtggtggccatcgccagccacgatggcggcaagcaggcgctggagacggtccagcggctgttgccggtgctgtgccaggcccacggcttgaccccggagcaggtggtggccatcgccagcaatattggtggcaagcaggcgctggagacggtgcaggcgctgttgccggtgctgtgccaggcccacggcttgaccccccagcaggtggtggccatcgccagcaataatggtggcaagcaggcgctggagacggtccagcggctgttgccggtgctgtgccaggcccacggcttgaccccccagcaggtggtggccatcgccagcaatggcggtggcaagcaggcgctggagacggtccagcggctgttgccggtgctgtgccaggcccacggcttgaccccggagcaggtggtggccatcgccagcaatattggtggcaagcaggcgctggagacggtgcaggcgctgttgccggtgctgtgccaggcccacggcttgaccccggagcaggtggtggccatcgccagccacgatggcggcaagcaggcgctggagacggtccagcggctgttgccggtgctgtgccaggcccacggcttgaccccggagcaggtggtggccatcgccagccacgatggcggcaagcaggcgctggagacggtccagcggctgttgccggtgctgtgccaggcccacggcttgaccccggagcaggtggtggccatcgccagcaatattggtggcaagcaggcgctggagacggtgcaggcgctgttgccggtgctgtgccaggcccacggcttgaccccggagcaggtggtggccatcgccagccacgatggcggcaagcaggcgctggagacggtccagcggctgttgccggtgctgtgccaggcccacggcttgacccctcagcaggtggtggccatcgccagcaatggcggcggcaggccggcgctggagagcattgttgcccagttatctcgccctgatccggcgttggccgcgttgaccaacgaccacctcgtcgccttggcctgcctcggcgggcgtcctgcgctggatgcagtgaaaaagggattgggggatcctatcagccgttcccagctggtgaagtccgagctggaggagaagaaatccgagttgaggcacaagctgaagtacgtgccccacgagtacatcgagctgatcgagatcgcccggaacagcacccaggaccgtatcctggagatgaaggtgatggagttcttcatgaaggtgtacggctacaggggcaagcacctgggcggctccaggaagcccgacggcgccatctacaccgtgggctcccccatcgactacggcgtgatcgtggacaccaaggcctactccggcggctacaacctgcccatcggccaggccgacgaaatgcagaggtacgtggaggagaaccagaccaggaacaagcacatcaaccccaacgagtggtggaaggtgtacccctccagcgtgaccgagttcaagttcctgttcgtgtccggccacttcaagggcaactacaaggcccagctgaccaggctgaaccacatcaccaactgcaacggcgccgtgctgtccgtggaggagctcctgatcggcggcgagatgatcaaggccggcaccctgaccctggaggaggtgaggaggaagttcaacaacggcgagatcaacttcgcggccgactgataa

SEQ ID NO: 95 - DNA, 2814 bp, Artificial sequence
  PDCD1_T01-L TALEN
atgggcgatcctaaaaagaaacgtaaggtcatcgattacccatacgatgttccagattacgctatcgatatcgccgatctacgcacgctcggctacagccagcagcaacaggagaagatcaaaccgaaggttcgttcgacagtggcgcagcaccacgaggcactggtcggccacgggtttacacacgcgcacatcgttgcgttaagccaacacccggcagcgttagggaccgtcgctgtcaagtatcaggacatgatcgcagcgttgccagaggcgacacacgaagcgatcgttggcgtcggcaaacagtggtccggcgcacgcgctctggaggccttgctcacggtggcgggagagttgagaggtccaccgttacagttggacacaggccaacttctcaagattgcaaaacgtggcggcgtgaccgcagtggaggcagtgcatgcatggcgcaatgcactgacgggtgccccgctcaacttgaccccccagcaggtggtggccatcgccagcaatggcggtggcaagcaggcgctggagacggtccagcggctgttgccggtgctgtgccaggcccacggcttgaccccggagcaggtggtggccatcgccagccacgatggcggcaagcaggcgctggagacggtccagcggctgttgccggtgctgtgccaggcccacggcttgaccccccagcaggtggtggccatcgccagcaatggcggtggcaagcaggcgctggagacggtccagcggctgttgccggtgctgtgccaggcccacggcttgaccccggagcaggtggtggccatcgccagccacgatggcggcaagcaggcgctggagacggtccagcggctgttgccggtgctgtgccaggcccacggcttgaccccggagcaggtggtggccatcgccagccacgatggcggcaagcaggcgctggagacggtccagcggctgttgccggtgctgtgccaggcccacggcttgaccccggagcaggtggtggccatcgccagccacgatggcggcaagcaggcgctggagacggtccagcggctgttgccggtgctgtgccaggcccacggcttgaccccggagcaggtggtggccatcgccagccacgatggcggcaagcaggcgctggagacggtccagcggctgttgccggtgctgtgccaggcccacggcttgaccccggagcaggtggtggccatcgccagcaatattggtggcaagcaggcgctggagacggtgcaggcgctgttgccggtgctgtgccaggcccacggcttgaccccccagcaggtggtggccatcgccagcaataatggtggcaagcaggcgctggagacggtccagcggctgttgccggtgctgtgccaggcccacggcttgaccccggagcaggtggtggccatcgccagccacgatggcggcaagcaggcgctggagacggtccagcggctgttgccggtgctgtgccaggcccacggcttgaccccggagcaggtggtggccatcgccagccacgatggcggcaagcaggcgctggagacggtccagcggctgttgccggtgctgtgccaggcccacggcttgaccccggagcaggtggtggccatcgccagccacgatggcggcaagcaggcgctggagacggtccagcggctgttgccggtgctgtgccaggcccacggcttgaccccccagcaggtggtggccatcgccagcaatggcggtggcaagcaggcgctggagacggtccagcggctgttgccggtgctgtgccaggcccacggcttgaccccccagcaggtggtggccatcgccagcaataatggtggcaagcaggcgctggagacggtccagcggctgttgccggtgctgtgccaggcccacggcttgaccccggagcaggtggtggccatcgccagccacgatggcggcaagcaggcgctggagacggtccagcggctgttgccggtgctgtgccaggcccacggcttgacccctcagcaggtggtggccatcgccagcaatggcggcggcaggccggcgctggagagcattgttgcccagttatctcgccctgatccggcgttggccgcgttgaccaacgaccacctcgtcgccttggcctgcctcggcgggcgtcctgcgctggatgcagtgaaaaagggattgggggatcctatcagccgttcccagctggtgaagtccgagctggaggagaagaaatccgagttgaggcacaagctgaagtacgtgccccacgagtacatcgagctgatcgagatcgcccggaacagcacccaggaccgtatcctggagatgaaggtgatggagttcttcatgaaggtgtacggctacaggggcaagcacctgggcggctccaggaagcccgacggcgccatctacaccgtgggctcccccatcgactacggcgtgatcgtggacaccaaggcctactccggcggctacaacctgcccatcggccaggccgacgaaatgcagaggtacgtggaggagaaccagaccaggaacaagcacatcaaccccaacgagtggtggaaggtgtacccctccagcgtgaccgagttcaagttcctgttcgtgtccggccacttcaagggcaactacaaggcccagctgaccaggctgaaccacatcaccaactgcaacggcgccgtgctgtccgtggaggagctcctgatcggcggcgagatgatcaaggccggcaccctgaccctggaggaggtgaggaggaagttcaacaacggcgagatcaacttcgcggccgactgataa

SEQ ID NO: 96 - DNA, 2829 bp, Artificial sequence
  PDCD1_T01-R TALEN
atgggcgatcctaaaaagaaacgtaaggtcatcgataaggagaccgccgctgccaagttcgagagacagcacatggacagcatcgatatcgccgatctacgcacgctcggctacagccagcagcaacaggagaagatcaaaccgaaggttcgttcgacagtggcgcagcaccacgaggcactggtcggccacgggtttacacacgcgcacatcgttgcgttaagccaacacccggcagcgttagggaccgtcgctgtcaagtatcaggacatgatcgcagcgttgccagaggcgacacacgaagcgatcgttggcgtcggcaaacagtggtccggcgcacgcgctctggaggccttgctcacggtggcgggagagttgagaggtccaccgttacagttggacacaggccaacttctcaagattgcaaaacgtggcggcgtgaccgcagtggaggcagtgcatgcatggcgcaatgcactgacgggtgccccgctcaacttgaccccccagcaagtcgtcgcaatcgccagcaataacggagggaagcaagccctcgaaaccgtgcagcggttgcttcctgtgctctgccaggcccacggccttacccctgagcaggtggtggccatcgcaagtaacattggaggaaagcaagccttggagacagtgcaggccctgttgcccgtgctgtgccaggcacacggcctcacaccagagcaggtcgtggccattgcctccaacatcggggggaaacaggctctggagaccgtccaggccctgctgcccgtcctctgtcaagctcacggcctgactccccaacaagtggtcgccatcgcctctaataacggcgggaagcaggcactggaaacagtgcagagactgctccctgtgctttgccaagctcatgggttgaccccccaacaggtcgtcgctattgcctcaaacaacgggggcaagcaggcccttgagactgtgcagaggctgttgccagtgctgtgtcaggctcacgggctcactccacaacaggtggtcgcaattgccagcaacggcggcggaaagcaagctcttgaaaccgtgcaacgcctcctgcccgtgctctgtcaggctcatggcctgacaccacaacaagtcgtggccatcgccagtaataatggcgggaaacaggctcttgagaccgtccagaggctgctcccagtgctctgccaggcacacgggctgaccccccagcaggtggtggctatcgccagcaataatgggggcaagcaggccctggaaacagtccagcgcctgctgccagtgctttgccaggctcacgggctcactcccgaacaggtcgtggcaatcgcctccaacggagggaagcaggctctggagaccgtgcagagactgctgcccgtcttgtgccaggcccacggactcacacctcagcaggtcgtcgccattgcctctaacaacgggggcaaacaagccctggagacagtgcagcggctgttgcctgtgttgtgccaagcccacggcttgactcctcaacaagtggtcgccatcgcctcaaatggcggcggaaaacaagctctggagacagtgcagaggttgctgcccgtcctctgccaagcccacggcctgactccccaacaggtcgtcgccattgccagcaacggcggaggaaagcaggctctcgaaactgtgcagcggctgcttcctgtgctgtgtcaggctcatgggctgaccccccagcaagtggtggctattgcctctaacaatggaggcaagcaagcccttgagacagtccagaggctgttgccagtgctgtgccaggcccacgggctcacaccccagcaggtggtcgccatcgccagtaacggcgggggcaaacaggcattggaaaccgtccagcgcctgcttccagtgctctgccaggcacacggactgacacccgaacaggtggtggccattgcatcccatgatgggggcaagcaggccctggagaccgtgcagagactcctgccagtgttgtgccaagctcacggcctcacccctcagcaagtcgtggccatcgcctcaaacggggggggccggcctgcactggagagcattgttgcccagttatctcgccctgatccggcgttggccgcgttgaccaacgaccacctcgtcgccttggcctgcctcggcgggcgtcctgcgctggatgcagtgaaaaagggattgggggatcctatcagccgttcccagctggtgaagtccgagctggaggagaagaaatccgagttgaggcacaagctgaagtacgtgccccacgagtacatcgagctgatcgagatcgcccggaacagcacccaggaccgtatcctggagatgaaggtgatggagttcttcatgaaggtgtacggctacaggggcaagcacctgggcggctccaggaagcccgacggcgccatctacaccgtgggctcccccatcgactacggcgtgatcgtggacaccaaggcctactccggcggctacaacctgcccatcggccaggccgacgaaatgcagaggtacgtggaggagaaccagaccaggaacaagcacatcaaccccaacgagtggtggaaggtgtacccctccagcgtgaccgagttcaagttcctgttcgtgtccggccacttcaagggcaactacaaggcccagctgaccaggctgaaccacatcaccaactgcaacggcgccgtgctgtccgtggaggagctcctgatcggcggcgagatgatcaaggccggcaccctgaccctggaggaggtgaggaggaagttcaacaacggcgagatcaacttcgcggccgactgataa

SEQ ID NO: 97 - DNA, 2814 bp, Artificial sequence
  PDCD1_T03-L TALEN
atgggcgatcctaaaaagaaacgtaaggtcatcgattacccatacgatgttccagattacgctatcgatatcgccgatctacgcacgctcggctacagccagcagcaacaggagaagatcaaaccgaaggttcgttcgacagtggcgcagcaccacgaggcactggtcggccacgggtttacacacgcgcacatcgttgcgttaagccaacacccggcagcgttagggaccgtcgctgtcaagtatcaggacatgatcgcagcgttgccagaggcgacacacgaagcgatcgttggcgtcggcaaacagtggtccggcgcacgcgctctggaggccttgctcacggtggcgggagagttgagaggtccaccgttacagttggacacaggccaacttctcaagattgcaaaacgtggcggcgtgaccgcagtggaggcagtgcatgcatggcgcaatgcactgacgggtgccccgctcaacttgaccccggagcaggtggtggccatcgccagcaatattggtggcaagcaggcgctggagacggtgcaggcgctgttgccggtgctgtgccaggcccacggcttgaccccggagcaggtggtggccatcgccagccacgatggcggcaagcaggcgctggagacggtccagcggctgttgccggtgctgtgccaggcccacggcttgaccccggagcaggtggtggccatcgccagccacgatggcggcaagcaggcgctggagacggtccagcggctgttgccggtgctgtgccaggcccacggcttgaccccccagcaggtggtggccatcgccagcaatggcggtggcaagcaggcgctggagacggtccagcggctgttgccggtgctgtgccaggcccacggcttgaccccggagcaggtggtggccatcgccagccacgatggcggcaagcaggcgctggagacggtccagcggctgttgccggtgctgtgccaggcccacggcttgaccccccagcaggtggtggccatcgccagcaatggcggtggcaagcaggcgctggagacggtccagcggctgttgccggtgctgtgccaggcccacggcttgaccccccagcaggtggtggccatcgccagcaataatggtggcaagcaggcgctggagacggtccagcggctgttgccggtgctgtgccaggcccacggcttgaccccccagcaggtggtggccatcgccagcaatggcggtggcaagcaggcgctggagacggtccagcggctgttgccggtgctgtgccaggcccacggcttgaccccccagcaggtggtggccatcgccagcaataatggtggcaagcaggcgctggagacggtccagcggctgttgccggtgctgtgccaggcccacggcttgaccccccagcaggtggtggccatcgccagcaataatggtggcaagcaggcgctggagacggtccagcggctgttgccggtgctgtgccaggcccacggcttgaccccccagcaggtggtggccatcgccagcaataatggtggcaagcaggcgctggagacggtccagcggctgttgccggtgctgtgccaggcccacggcttgaccccccagcaggtggtggccatcgccagcaataatggtggcaagcaggcgctggagacggtccagcggctgttgccggtgctgtgccaggcccacggcttgaccccggagcaggtggtggccatcgccagccacgatggcggcaagcaggcgctggagacggtccagcggctgttgccggtgctgtgccaggcccacggcttgaccccggagcaggtggtggccatcgccagccacgatggcggcaagcaggcgctggagacggtccagcggctgttgccggtgctgtgccaggcccacggcttgaccccggagcaggtggtggccatcgccagcaatattggtggcaagcaggcgctggagacggtgcaggcgctgttgccggtgctgtgccaggcccacggcttgacccctcagcaggtggtggccatcgccagcaatggcggcggcaggccggcgctggagagcattgttgcccagttatctcgccctgatccggcgttggccgcgttgaccaacgaccacctcgtcgccttggcctgcctcggcgggcgtcctgcgctggatgcagtgaaaaagggattgggggatcctatcagccgttcccagctggtgaagtccgagctggaggagaagaaatccgagttgaggcacaagctgaagtacgtgccccacgagtacatcgagctgatcgagatcgcccggaacagcacccaggaccgtatcctggagatgaaggtgatggagttcttcatgaaggtgtacggctacaggggcaagcacctgggcggctccaggaagcccgacggcgccatctacaccgtgggctcccccatcgactacggcgtgatcgtggacaccaaggcctactccggcggctacaacctgcccatcggccaggccgacgaaatgcagaggtacgtggaggagaaccagaccaggaacaagcacatcaaccccaacgagtggtggaaggtgtacccctccagcgtgaccgagttcaagttcctgttcgtgtccggccacttcaagggcaactacaaggcccagctgaccaggctgaaccacatcaccaactgcaacggcgccgtgctgtccgtggaggagctcctgatcggcggcgagatgatcaaggccggcaccctgaccctggaggaggtgaggaggaagttcaacaacggcgagatcaacttcgcggccgactgataa

SEQ ID NO: 98 - DNA, 2829 bp, Artificial sequence
  PDCD1_T03-R TALEN
atgggcgatcctaaaaagaaacgtaaggtcatcgataaggagaccgccgctgccaagttcgagagacagcacatggacagcatcgatatcgccgatctacgcacgctcggctacagccagcagcaacaggagaagatcaaaccgaaggttcgttcgacagtggcgcagcaccacgaggcactggtcggccacgggtttacacacgcgcacatcgttgcgttaagccaacacccggcagcgttagggaccgtcgctgtcaagtatcaggacatgatcgcagcgttgccagaggcgacacacgaagcgatcgttggcgtcggcaaacagtggtccggcgcacgcgctctggaggccttgctcacggtggcgggagagttgagaggtccaccgttacagttggacacaggccaacttctcaagattgcaaaacgtggcggcgtgaccgcagtggaggcagtgcatgcatggcgcaatgcactgacgggtgccccgctcaacttgacccccgagcaagtcgtcgcaatcgccagccatgatggagggaagcaagccctcgaaaccgtgcagcggttgcttcctgtgctctgccaggcccacggccttacccctcagcaggtggtggccatcgcaagtaacggaggaggaaagcaagccttggagacagtgcagcgcctgttgcccgtgctgtgccaggcacacggcctcacaccagagcaggtcgtggccattgcctcccatgacggggggaaacaggctctggagaccgtccagaggctgctgcccgtcctctgtcaagctcacggcctgactccccaacaagtggtcgccatcgcctctaatggcggcgggaagcaggcactggaaacagtgcagagactgctccctgtgctttgccaagctcatgggttgaccccccaacaggtcgtcgctattgcctcaaacggggggggcaagcaggcccttgagactgtgcagaggctgttgccagtgctgtgtcaggctcacgggctcactccacaacaggtggtcgcaattgccagcaacggcggcggaaagcaagctcttgaaaccgtgcaacgcctcctgcccgtgctctgtcaggctcatggcctgacaccacaacaagtcgtggccatcgccagtaataatggcgggaaacaggctcttgagaccgtccagaggctgctcccagtgctctgccaggcacacgggctgacccccgagcaggtggtggctatcgccagcaatattgggggcaagcaggccctggaaacagtccaggccctgctgccagtgctttgccaggctcacgggctcactccccagcaggtcgtggcaatcgcctccaacggcggagggaagcaggctctggagaccgtgcagagactgctgcccgtcttgtgccaggcccacggactcacacctgaacaggtcgtcgccattgcctctcacgatgggggcaaacaagccctggagacagtgcagcggctgttgcctgtgttgtgccaagcccacggcttgactcctcaacaagtggtcgccatcgcctcaaatggcggcggaaaacaagctctggagacagtgcagaggttgctgcccgtcctctgccaagcccacggcctgactccccaacaggtcgtcgccattgccagcaacaacggaggaaagcaggctctcgaaactgtgcagcggctgcttcctgtgctgtgtcaggctcatgggctgacccccgagcaagtggtggctattgcctctaatggaggcaagcaagcccttgagacagtccagaggctgttgccagtgctgtgccaggcccacgggctcacaccccagcaggtggtcgccatcgccagtaacaacgggggcaaacaggcattggaaaccgtccagcgcctgcttccagtgctctgccaggcacacggactgacacccgaacaggtggtggccattgcatcccatgatgggggcaagcaggccctggagaccgtgcagagactcctgccagtgttgtgccaagctcacggcctcacccctcagcaagtcgtggccatcgcctcaaacggggggggccggcctgcactggagagcattgttgcccagttatctcgccctgatccggcgttggccgcgttgaccaacgaccacctcgtcgccttggcctgcctcggcgggcgtcctgcgctggatgcagtgaaaaagggattgggggatcctatcagccgttcccagctggtgaagtccgagctggaggagaagaaatccgagttgaggcacaagctgaagtacgtgccccacgagtacatcgagctgatcgagatcgcccggaacagcacccaggaccgtatcctggagatgaaggtgatggagttcttcatgaaggtgtacggctacaggggcaagcacctgggcggctccaggaagcccgacggcgccatctacaccgtgggctcccccatcgactacggcgtgatcgtggacaccaaggcctactccggcggctacaacctgcccatcggccaggccgacgaaatgcagaggtacgtggaggagaaccagaccaggaacaagcacatcaaccccaacgagtggtggaaggtgtacccctccagcgtgaccgagttcaagttcctgttcgtgtccggccacttcaagggcaactacaaggcccagctgaccaggctgaaccacatcaccaactgcaacggcgccgtgctgtccgtggaggagctcctgatcggcggcgagatgatcaaggccggcaccctgaccctggaggaggtgaggaggaagttcaacaacggcgagatcaacttcgcggccgactgataa

SEQ ID NO: 99 - DNA, 60 bp, Artificial sequence
  Forward primer CTLA4_T01
  misc_feature (31); (32); (33); (34); (35); (36); (37); (38); (39); (40): n is a or c or t or g
ccatctcatccctgcgtgtctccgactcagnnnnnnnnnnctctacttcctgaagacctg

SEQ ID NO: 100 - DNA, 60 bp, Artificial sequence
  Forward primer CTLA4_T03/T04
  misc_feature (31); (32); (33); (34); (35); (36); (37); (38); (39); (40): n is a or c or t or g
ccatctcatccctgcgtgtctccgactcagnnnnnnnnnnacagttgagagatggagggg

SEQ ID NO: 101 - DNA, 59 bp, Artificial sequence
  Forward primer PDCD1_T01
  misc_feature (31); (32); (33); (34); (35); (36); (37); (38); (39); (40): n is a or c or t or g
ccatctcatccctgcgtgtctccgactcagnnnnnnnnnnccacagaggtaggtgccgc

SEQ ID NO: 102 - DNA, 60 bp, Artificial sequence
  Forward primer PDCD1_T03
  misc_feature (31); (32); (33); (34); (35); (36); (37); (38); (39); (40): n is a or c or t or g
ccatctcatccctgcgtgtctccgactcagnnnnnnnnnngacagagatgccggtcacca

SEQ ID NO: 103 - DNA, 50 bp, Artificial sequence
  Reverse primer CTLA4_T01
cctatcccctgtgtgccttggcagtctcagtggaatacagagccagccaa

SEQ ID NO: 104 - DNA, 50 bp, Artificial sequence
  Reverse primer CTLA4_T03/04
cctatcccctgtgtgccttggcagtctcagggtgcccgtgcagatggaat

SEQ ID NO: 105 - DNA, 50 bp, Artificial sequence
  Reverse primer PDCD1_T01
cctatcccctgtgtgccttggcagtctcagggctctgcagtggaggccag

SEQ ID NO: 106 - DNA, 50 bp, Artificial sequence
  Reverse primer PDCD1_T03
cctatcccctgtgtgccttggcagtctcagggacaacgccaccttcacct

SEQ ID NO: 107 - protein, 281 aa, Artificialsequence
  pTalpha-FL
MAGTWLLLLLALGCPALPTGVGGTPFPSLAPPIMLLVDGKQQMVVVCLVLDVAPPGLDSPIWFSAGNGSALDAFTYGPSPATDGTWTNLAHLSLPSEELASWEPLVCHTGPGAEGHSRSTQPMHLSGEASTARTCPQEPLRGTPGGALWLGVLRLLLFKLLLFDLLLTCSCLCDPAGPLPSPATTTRLRALGSHRLHPATETGGREATSSPRPQPRDRRWGDTPPGRKPGSPVWGEGSYLSSYPTCPAQAWCSRSRLRAPSSSLGAFFRGDLPPPLQAGAA

SEQ ID NO: 108 - protein, 263 aa, Artificialsequence
  pTalpha-Delta18
MAGTWLLLLLALGCPALPTGVGGTPFPSLAPPIMLLVDGKQQMVVVCLVLDVAPPGLDSPIWFSAGNGSALDAFTYGPSPATDGTWTNLAHLSLPSEELASWEPLVCHTGPGAEGHSRSTQPMHLSGEASTARTCPQEPLRGTPGGALWLGVLRLLLFKLLLFDLLLTCSCLCDPAGPLPSPATTTRLRALGSHRLHPATETGGREATSSPRPQPRDRRWGDTPPGRKPGSPVWGEGSYLSSYPTCPAQAWCSRSRLRAPSSS

SEQ ID NO: 109 - protein, 233 aa, Artificialsequence
  pTalpha-Delta48
MAGTWLLLLLALGCPALPTGVGGTPFPSLAPPIMLLVDGKQQMVVVCLVLDVAPPGLDSPIWFSAGNGSALDAFTYGPSPATDGTWTNLAHLSLPSEELASWEPLVCHTGPGAEGHSRSTQPMHLSGEASTARTCPQEPLRGTPGGALWLGVLRLLLFKLLLFDLLLTCSCLCDPAGPLPSPATTTRLRALGSHRLHPATETGGREATSSPRPQPRDRRWGDTPPGRKPGSPV

SEQ ID NO: 110 - protein, 219 aa, Artificialsequence
  pTalpha-Delta62
MAGTWLLLLLALGCPALPTGVGGTPFPSLAPPIMLLVDGKQQMVVVCLVLDVAPPGLDSPIWFSAGNGSALDAFTYGPSPATDGTWTNLAHLSLPSEELASWEPLVCHTGPGAEGHSRSTQPMHLSGEASTARTCPQEPLRGTPGGALWLGVLRLLLFKLLLFDLLLTCSCLCDPAGPLPSPATTTRLRALGSHRLHPATETGGREATSSPRPQPRDRR

SEQ ID NO: 111 - protein, 203 aa, Artificialsequence
  pTalpha-Delta78
MAGTWLLLLLALGCPALPTGVGGTPFPSLAPPIMLLVDGKQQMVVVCLVLDVAPPGLDSPIWFSAGNGSALDAFTYGPSPATDGTWTNLAHLSLPSEELASWEPLVCHTGPGAEGHSRSTQPMHLSGEASTARTCPQEPLRGTPGGALWLGVLRLLLFKLLLFDLLLTCSCLCDPAGPLPSPATTTRLRALGSHRLHPATETG

SEQ ID NO: 112 - protein, 189 aa, Artificialsequence
  pTalpha-Delta92
MAGTWLLLLLALGCPALPTGVGGTPFPSLAPPIMLLVDGKQQMVVVCLVLDVAPPGLDSPIWFSAGNGSALDAFTYGPSPATDGTWTNLAHLSLPSEELASWEPLVCHTGPGAEGHSRSTQPMHLSGEASTARTCPQEPLRGTPGGALWLGVLRLLLFKLLLFDLLLTCSCLCDPAGPLPSPATTTRLR

SEQ ID NO: 113 - protein, 171 aa, Artificialsequence
  pTalpha-Delta110
MAGTWLLLLLALGCPALPTGVGGTPFPSLAPPIMLLVDGKQQMVVVCLVLDVAPPGLDSPIWFSAGNGSALDAFTYGPSPATDGTWTNLAHLSLPSEELASWEPLVCHTGPGAEGHSRSTQPMHLSGEASTARTCPQEPLRGTPGGALWLGVLRLLLFKLLLFDLLLTCSC

SEQ ID NO: 114 - protein, 167 aa, Artificialsequence
  pTalpha-Delta114
MAGTWLLLLLALGCPALPTGVGGTPFPSLAPPIMLLVDGKQQMVVVCLVLDVAPPGLDSPIWFSAGNGSALDAFTYGPSPATDGTWTNLAHLSLPSEELASWEPLVCHTGPGAEGHSRSTQPMHLSGEASTARTCPQEPLRGTPGGALWLGVLRLLLFKLLLFDLLL

SEQ ID NO: 115 - protein, 344 aa, Artificialsequence [sequence omitted]

SEQ ID NO: 116 - protein, 311 aa, Artificialsequence
  pTalpha-FL-CD8
MAGTWLLLLLALGCPALPTGVGGTPFPSLAPPIMLLVDGKQQMVVVCLVLDVAPPGLDSPIWFSAGNGSALDAFTYGPSPATDGTWTNLAHLSLPSEELASWEPLVCHTGPGAEGHSRSTQPMHLSGEASTARTCPQEPLRGTPGGALWLGVLRLLLFKLLLFDLLLTCSCLCDPAGPLPSPATTTRLRALGSHRLHPATETGGREATSSPRPQPRDRRWGDTPPGRKPGSPVWGEGSYLSSYPTCPAQAWCSRSRLRAPSSSLGAFFRGDLPPPLQAGAAASHRNRRRVCKCPRPVVKSGDKPSLSARYV

SEQ ID NO: 117 - protein, 325 aa, Artificialsequence
  pTalpha-FL-41BB
MAGTWLLLLLALGCPALPTGVGGTPFPSLAPPIMLLVDGKQQMVVVCLVLDVAPPGLDSPIWFSAGNGSALDAFTYGPSPATDGTWTNLAHLSLPSEELASWEPLVCHTGPGAEGHSRSTQPMHLSGEASTARTCPQEPLRGTPGGALWLGVLRLLLFKLLLFDLLLTCSCLCDPAGPLPSPATTTRLRALGSHRLHPATETGGREATSSPRPQPRDRRWGDTPPGRKPGSPVWGEGSYLSSYPTCPAQAWCSRSRLRAPSSSLGAFFRGDLPPPLQAGAAGSKRGRKKLLYIFKQPFMRPVQTTQEEDGCSCRFPEEEEGGCEL

SEQ ID NO: 118 - protein, 296 aa, Artificialsequence
  pTalpha-Delta48-CD28
MAGTWLLLLLALGCPALPTGVGGTPFPSLAPPIMLLVDGKQQMVVVCLVLDVAPPGLDSPIWFSAGNGSALDAFTYGPSPATDGTWTNLAHLSLPSEELASWEPLVCHTGPGAEGHSRSTQPMHLSGEASTARTCPQEPLRGTPGGALWLGVLRLLLFKLLLFDLLLTCSCLCDPAGPLPSPATTTRLRALGSHRLHPATETGGREATSSPRPQPRDRRWGDTPPGRKPGSPVASGGVLACYSLLVTVAFIIFWVRSKRSRGGHSDYMNMTPRRPGPTRKHYQPYAPPRDFAAYRS

SEQ ID NO: 119 - protein, 263 aa, Artificialsequence
  pTalpha-Delta48-CD8
MAGTWLLLLLALGCPALPTGVGGTPFPSLAPPIMLLVDGKQQMVVVCLVLDVAPPGLDSPIWFSAGNGSALDAFTYGPSPATDGTWTNLAHLSLPSEELASWEPLVCHTGPGAEGHSRSTQPMHLSGEASTARTCPQEPLRGTPGGALWLGVLRLLLFKLLLFDLLLTCSCLCDPAGPLPSPATTTRLRALGSHRLHPATETGGREATSSPRPQPRDRRWGDTPPGRKPGSPVASHRNRRRVCKCPRPVVKSGDKPSLSARYV

SEQ ID NO: 120 - protein, 277 aa, Artificialsequence
  pTalpha-Delta48-41BB
MAGTWLLLLLALGCPALPTGVGGTPFPSLAPPIMLLVDGKQQMVVVCLVLDVAPPGLDSPIWFSAGNGSALDAFTYGPSPATDGTWTNLAHLSLPSEELASWEPLVCHTGPGAEGHSRSTQPMHLSGEASTARTCPQEPLRGTPGGALWLGVLRLLLFKLLLFDLLLTCSCLCDPAGPLPSPATTTRLRALGSHRLHPATETGGREATSSPRPQPRDRRWGDTPPGRKPGSPVGSKRGRKKLLYIFKQPFMRPVQTTQEEDGCSCRFPEEEEGGCEL

SEQ ID NO: 121 - protein, 172 aa, Artificialsequence
  pTalpha-Delta114-TCRalpha.IC
MAGTWLLLLLALGCPALPTGVGGTPFPSLAPPIMLLVDGKQQMVVVCLVLDVAPPGLDSPIWFSAGNGSALDAFTYGPSPATDGTWTNLAHLSLPSEELASWEPLVCHTGPGAEGHSRSTQPMHLSGEASTARTCPQEPLRGTPGGALWLGVLRLLLFKLLLFDLLLRLWSS

SEQ ID NO: 122 - protein, 173 aa, Artificialsequence
  pTalpha.EC-TCRalpha. TM. IC
MAGTWLLLLLALGCPALPTGVGGTPFPSLAPPIMLLVDGKQQMVVVCLVLDVAPPGLDSPIWFSAGNGSALDAFTYGPSPATDGTWTNLAHLSLPSEELASWEPLVCHTGPGAEGHSRSTQPMHLSGEASTARTCPQEPLRGTPGGLSVIGFRILLLKVAGFNLLMTLRLWSS

SEQ ID NO: 123 - protein, 233 aa, Artificialsequence
  pTalpha.EC-Delta48-1xMUT
MAGTWLLLLLALGCPALPTGVGGTPFPSLAPPIMLLVDGKQQMVVVCLVLDVAPPGLDSPIRFSAGNGSALDAFTYGPSPATDGTWTNLAHLSLPSEELASWEPLVCHTGPGAEGHSRSTQPMHLSGEASTARTCPQEPLRGTPGGALWLGVLRLLLFKLLLFDLLLTCSCLCDPAGPLPSPATTTRLRALGSHRLHPATETGGREATSSPRPQPRDRRWGDTPPGRKPGSPV

SEQ ID NO: 124 - protein, 233 aa, Artificialsequence
  pTalpha.EC-Delta48-4xMUT
MAGTWLLLLLALGCPALPTGVGGTPFPSLAPPIMLLVAGAQQMVVVCLVLDVAPPGLDSPIWFSAGNGSALDAFTYGPSPATDGTWTNLAHLSLPSEELASWEPLVCHTGPGAEGHSASTQPMHLSGEASTAATCPQEPLRGTPGGALWLGVLRLLLFKLLLFDLLLTCSCLCDPAGPLPSPATTTRLRALGSHRLHPATETGGREATSSPRPQPRDRRWGDTPPGRKPGSPV

SEQ ID NO: 125 - protein, 848 aa, Artificialsequence
  Multi-chain CAR
MAPAMESPTLLCVALLFFAPDGVLAEVQLQQSGPELIKPGASVKMSCKASGYTFTSYVMHWVKQKPGQGLEWIGYINPYNDGTKYNEKFKGKATLTSDKSSSTAYMELSSLTSEDSAVYYCARGTYYYGSRVFDYWGQGTTLTVSSGGGGSGGGGSGGGGSDIVMTQAAPSIPVTPGESVSISCRSSKSLLNSNGNTYLYWFLQRPGQSPQLLIYRMSNLASGVPDRFSGSGSGTAFTLRISRVEAEDVGVYYCMQHLEYPFTFGAGTKLELKRADTTTPAPRPPTPAPTIASQPLSLRPEACRPAAGGAVHTRGLDFACDFFIPLLVVILFAVDTGLFISTQQQVTFLLKIKRTRKGFRLLNPHPKPNPKNNRAEGRGSLLTCGDVEENPGPMDTESNRRANLALPQEPSSVPAFEVLEISPQEVSSGRLLKSASSPPLHTWLTVLKKEQEFLGVTQILTAMICLCFGTVVCSVLDISHIEGDIFSSFKAGYPFWGAIFFSISGMLSIISERRNATYLVRGSLGANTASSIAGGTGITILIINLKKSLAYIHIHSCQKFFETKCFMASFSTEIVVMMLFLTILGLGSAVSLTICGAGEELKGNKVPEKRGRKKLLYIFKQPFMRPVQTTQEEDGCSCRFPEEEEGGCELGSGVKQTLNFDLLKLAGDVESNPGPMIPAVVLLLLLLVEQAAALGEPQLCYILDAILFLYGIVLTLLYCRLKIQVRKAAITSYEKSRVKFSRSADAPAYQQGQNQLYNELNLGRREEYDVLDKRRGRDPEMGGKPRRKNPQEGLYNELQKDKMAEAYSEIGMKGERRRGKGHDGLYQGLSTATKDTYDALHMQALPPR

SEQ ID NO: 126 - DNA, 2547 bp, Artificialsequence
  Multi-chain CAR
atggctcctgccatggaatcccctactctactgtgtgtagccttactgttcttcgctccagatggcgtgttagcagaggtgcagttgcagcagtcagggccagagttgattaagcccggagcctccgtcaagatgtcctgcaaggccagcgggtacactttcaccagctacgtcatgcattgggtgaagcagaagccaggccaggggcttgagtggattgggtacatcaacccctacaacgacgggaccaaatacaacgagaaattcaagggcaaagccacactcacctccgataagtcctcctctaccgcctacatggagctcagctccctgacctccgaggatagcgctgtgtattactgcgcaaggggcacatactactatggctctagggtgttcgactactgggggcagggcactactctcacagtgagctcaggcggaggaggcagtggcggagggggaagtgggggcggcggcagcgatattgtcatgacccaggcagcccctagtatccctgtgactccaggcgagagcgtgagcatcagctgccggtccagcaagagcctgctgaacagtaacggaaacacatacctctactggtttctgcagaggcccggccagagccctcagctgctgatttaccgcatgtcaaatcttgcctctggggtgcccgatagatttagtgggagcggatccggcacagcttttacattgcggatctccagagtcgaggccgaagacgtgggggtctattactgtatgcaacacctggaatacccctttaccttcggagccggcacaaagctggagctgaagcgggctgacaccacaacccccgctccaaggccccctacccccgcaccaactattgcctcccagccactctcactgcggcctgaggcctgtcggcccgctgctggaggcgcagtgcatacaaggggcctcgatttcgcctgcgatttttttatcccattgttggtggtgattctgtttgctgtggacacaggattatttatctcaactcagcagcaggtcacatttctcttgaagattaagagaaccaggaaaggcttcagacttctgaacccacatcctaagccaaaccccaaaaacaacagagccgagggcagaggcagcctgctgacctgcggcgacgtggaggagaacccaggccccatggacacagaaagtaataggagagcaaatcttgctctcccacaggagccttccagtgtgcctgcatttgaagtcttggaaatatctccccaggaagtatcttcaggcagactattgaagtcggcctcatccccaccactgcatacatggctgacagttttgaaaaaagagcaggagttcctgggggtaacacaaattctgactgctatgatatgcctttgttttggaacagttgtctgctctgtacttgatatttcacacattgagggagacattttttcatcatttaaagcaggttatccattctggggagccatatttttttctatttctggaatgttgtcaattatatctgaaaggagaaatgcaacatatctggtgagaggaagcctgggagcaaacactgccagcagcatagctgggggaacgggaattaccatcctgatcatcaacctgaagaagagcttggcctatatccacatccacagttgccagaaattttttgagaccaagtgctttatggcttccttttccactgaaattgtagtgatgatgctgtttctcaccattctgggacttggtagtgctgtgtcactcacaatctgtggagctggggaagaactcaaaggaaacaaggttccagagaaacggggccggaagaagctcctctacatttttaagcagcctttcatgcggccagtgcagacaacccaagaggaggatgggtgttcctgcagattccctgaggaagaggaaggcgggtgcgagctgggttctggcgtgaaacagactttgaattttgaccttctcaagttggcgggagacgtggagtccaacccagggcccatgattccagcagtggtcttgctcttactccttttggttgaacaagcagcggccctgggagagcctcagctctgctatatcctggatgccatcctgtttctgtatggaattgtcctcaccctcctctactgtcgactgaagatccaagtgcgaaaggcagctataaccagctatgagaaatcaagagtgaagttctccaggagcgcagatgcccccgcctatcaacagggccagaaccagctctacaacgagcttaacctcgggaggcgcgaagaatacgacgtgttggataagagaagggggcgggaccccgagatgggaggaaagccccggaggaagaaccctcaggagggcctgtacaacgagctgcagaaggataagatggccgaggcctactcagagatcgggatgaagggggagcggcgccgcgggaaggggcacgatgggctctaccaggggctgagcacagccacaaaggacacatacgacgccttgcacatgcaggcccttccaccccggtga